European Patent Specification EP 3 456 820 B1, published June 19, 2024. Title: Neuartige 7beta-Hydroxysteroid Dehydrogenase-Mutanten und Verfahren zur Herstellung von Ursodesoxycholsäure. Applicant: PharmaZell GmbH. The sequence listing filed with the application follows.

SEQUENCE LISTING (69 sequences)

SEQ ID NO: 1 - DNA, 792 bp, Collinsella aerofaciens
  CDS (1)..(792)
atgaacctgagggagaagtacggtgagtggggcctgatcctgggcgcgaccgagggcgtcggcaaggcgttctgcgagaagatcgccgccggcggcatgaacgtcgtcatggtcggccgtcgcgaggagaagctgaacgtgctcgcaggcgagatccgcgagacctacggcgtggagaccaaggtcgtgcgcgccgactttagccagcccggcgctgccgagaccgtcttcgccgcgaccgagggcctggacatgggcttcatgagctacgtggcctgcctgcacagcttcggtaagatccaggacaccccctgggagaagcacgaggccatgatcaacgtcaacgtcgtgaccttcctcaagtgcttccaccactacatgcggatctttgccgcccaggaccgcggcgccgtgatcaacgtctcgtcgatgaccggcatcagctccagcccctggaacggccagtacggcgcgggcaaggccttcatcctcaagatgaccgaggccgtggcctgcgagtgcgagggcaccggcgtcgacgtcgaggtcatcaccctcggcaccaccctaacccccagcctgctgtccaacctccccggcggcccgcagggcgaggccgtcatgaagatcgccctcacccccgaggagtgcgttgacgaggcctttgagaagctgggtaaggagctctccgtcatcgccggccagcgcaacaaggactccgtccacgactggaaggcaaaccacaccgaggacgagtacatccgctacatggggtcgttctaccgcgactag

SEQ ID NO: 2 - protein, 263 aa, Collinsella aerofaciens
MNLREKYGEWGLILGATEGVGKAFCEKIAAGGMNVVMVGRREEKLNVLAGEIRETYGVETKVVRADFSQPGAAETVFAATEGLDMGFMSYVACLHSFGKIQDTPWEKHEAMINVNVVTFLKCFHHYMRIFAAQDRGAVINVSSMTGISSSPWNGQYGAGKAFILKMTEAVACECEGTGVDVEVITLGTTLTPSLLSNLPGGPQGEAVMKIALTPEECVDEAFEKLGKELSVIAGQRNKDSVHDWKANHTEDEYIRYMGSFYRD

SEQ ID NO: 3 - DNA, 31 bp, artificial
  PCR Primer
gggaattccatatgaacctgagggagaagta

SEQ ID NO: 4 - DNA, 27 bp, Artificial
  PCR Primer
cccaagcttctagtcgcggtagaacga

SEQ ID NO: 5 - DNA, 774 bp, Comamonas testosteroni
  CDS (1)..(774)
atgtccatcatcgtgataagcggctgcgccaccggcattggtgccgctacgcgcaaggtcctggaggcggccggtcaccagatcgtaggcatcgatatacgcgatgcggaagtgattgccgatctctcgacggccgaaggtcgaaagcaggcgattgccgatgtactggcgaagtgcagcaagggcatggacggcctggtgctgtgcgccggcctgggaccgcagaccaaggtgcttggcaatgtggtttcggtcaattattttggcgcgaccgagctgatggatgcctttttgccagcgctgaaaaaaggccatcagcccgcagccgtcgtcatctcgtccgtggcttccgcgcatctggcttttgacaagaacccactggcgctggcactggaagccggcgaggaagccaaggcccgcgccattgtcgaacatgcgggagagcagggcggaaatctggcctatgcgggcagcaagaatgctttgacggtggctgtgcgcaaacgcgccgccgcctggggcgaggctggcgtgcgcctgaacaccatcgcccccggtgcaaccgagactcccttgctgcaggcgggcctgcaggacccgcgctatggcgaatccattgccaagttcgttcctcccatgggccgccgtgccgagccgtccgagatggcgtcggtcatcgcctttttgatgagcccggccgcaagctatgtgcatggcgcgcagatcgtcattgatggcggcattgatgcggtgatgcgcccgacacagttctga

SEQ ID NO: 6 - protein, 257 aa, Comamonas testosteroni [sequence omitted]

SEQ ID NO: 7 - DNA, 969 bp, Rattus norvegicus
  CDS (1)..(969)
atggattccatatctctgcgtgtagcactaaatgatggtaacttcattcctgtactggggtttggaaccactgtgcctgagaaggttgctaaggatgaagttatcaaggctactaaaatagctatagataatggattccgccattttgactctgcttatttgtacgaagtagaagaggaagtgggccaagccattagaagcaagattgaagacggcactgtgaagagagaagatatattctatacttcaaagctttggagcactttccatagaccagagctggtccgaacttgcttggaaaagacactgaaaagcactcaactggactatgtggatctttatattattcatttcccaatggctttgcagcctggagatatatttttcccacgagatgagcatggaaaactattgtttgaaacagtggatatctgtgacacatgggaggccatggaaaagtgtaaggatgcaggattggccaagtctattggggtgtccaactttaactgcaggcagctggagaggattctgaataagccagggctcaaatacaagcctgtgtgcaaccaggtggaatgtcacctttatctcaaccagagcaaaatgctggactattgtaagtcaaaagacatcattctggtttcctactgcacgctgggaagttcacgagacaaaacatgggtggatcagaaaagtccagttctcctagatgatccagttctttgtgccatagcaaagaagtacaagcaaaccccagccctagttgcccttcgctaccagctgcagcgtggggttgtgcccctgatcaggagtttcaacgcgaagcggatcaaagagctaacacaggtttttgaattccagttggcttcagaggacatgaaagccctggatggcttgaacagaaatttcagatacaacaatgcaaaatattttgatgaccatcccaatcatccatttactgatgaatag

SEQ ID NO: 8 - protein, 322 aa, Rattus norvegicus
MDSISLRVALNDGNFIPVLGFGTTVPEKVAKDEVIKATKIAIDNGFRHFDSAYLYEVEEEVGQAIRSKIEDGTVKREDIFYTSKLWSTFHRPELVRTCLEKTLKSTQLDYVDLYIIHFPMALQPGDIFFPRDEHGKLLFETVDICDTWEAMEKCKDAGLAKSIGVSNFNCRQLERILNKPGLKYKPVCNQVECHLYLNQSKMLDYCKSKDIILVSYCTLGSSRDKTWVDQKSPVLLDDPVLCAIAKKYKQTPALVALRYQLQRGVVPLIRSFNAKRIKELTQVFEFQLASEDMKALDGLNRNFRYNNAKYFDDHPNHPFTDE

SEQ ID NO: 9 - DNA, 26 bp, Artificial
  PCR Primer
cgtcgtcatggtcgcccgtcgcgagg

SEQ ID NO: 10 - DNA, 26 bp, Artificial
  PCR Primer
cctcgcgacgggcgaccatgacgacg

SEQ ID NO: 11 - DNA, 26 bp, Artificial
  PCR Primer
cgtcgtcatggtcagccgtcgcgagg

SEQ ID NO: 12 - DNA, 26 bp, Artificial
  PCR Primer
cctcgcgacggctgaccatgacgacg

SEQ ID NO: 13 - DNA, 47 bp, Artificial
  PCR Primer
gcgaattcgtgaaaggagatatacatgaacctgagggagaagtacgg

SEQ ID NO: 14 - DNA, 1206 bp, Artificial
  Formiate Deydrogenase Mutant
  CDS (1)..(1206)
atggcaaaggtcctgtgcgttctttacgatgatccggtcgacggctacccgaagacctatgcccgcgacgatcttccgaagatcgaccactatccgggcggccagatcttgccgacgccgaaggccatcgacttcacgcccgggcagttgctcggctccgtctccggcgagctcggcctgcgcgaatatctcgaatccaacggccacaccctggtcgtgacctccgacaaggacggccccgactcggtgttcgagcgcgagctggtcgatgcggatgtcgtcatctcccagcccttctggccggcctatctgacgcccgagcgcatcgccaaggccaagaacctgaagctcgcgctcaccgccggcatcggttccgaccacgtcgatcttcagtcggctatcgaccgcaacgtcaccgtggcggaagtcacctactgcaactcgatcagcgtcgccgagcatgtggtgatgatgatcctgtcgctggtgcgcaactatctgccctcgcacgaatgggcgcggaagggcggctggaacatcgccgactgcgtctcccacgcctacgacctcgaggcgatgcatgtcggcaccgtggccgccggccgcatcggtctcgcggtgctgcgccgtctggcgccgttcgacgtgcacctgcactacaccggccgtcaccgcctgccggaatcggtcgagaaggagctcaacctcacctggcacgcgacccgcgaggacatgtatccggtttgcgacgtggtgacgctgaactgcccgctgcaccccgaaaccgagcacatgatcaatgacgagacgctgaagctgttcaagcgtggcgcctacatcgtcaacaccgcccgcggcaagctgtgcgaccgcgatgccgtggcacgtgcgctcgaatccggccggctggccggctatgccggcgacgtgtggttcccgcagccggcgccgaaggaccacccctggcggacgatgccctataacggcatgaccccgcacatctccggcaccacgctgaccgcgcaggcgcgttatgcggcgggcacccgcgagatcctggagtgcttcttcgagggccgtccgatccgcgacgaatacctcatcgtgcagggcggcgctcttgccggcaccggcgcgcattcctactcgaagggcaatgccaccggcggttcggaagaggccgccaagttcaagaaggcggtctga

SEQ ID NO: 15 - protein, 401 aa, Artificial
  Synthetic Construct
MAKVLCVLYDDPVDGYPKTYARDDLPKIDHYPGGQILPTPKAIDFTPGQLLGSVSGELGLREYLESNGHTLVVTSDKDGPDSVFERELVDADVVISQPFWPAYLTPERIAKAKNLKLALTAGIGSDHVDLQSAIDRNVTVAEVTYCNSISVAEHVVMMILSLVRNYLPSHEWARKGGWNIADCVSHAYDLEAMHVGTVAAGRIGLAVLRRLAPFDVHLHYTGRHRLPESVEKELNLTWHATREDMYPVCDVVTLNCPLHPETEHMINDETLKLFKRGAYIVNTARGKLCDRDAVARALESGRLAGYAGDVWFPQPAPKDHPWRTMPYNGMTPHISGTTLTAQARYAAGTREILECFFEGRPIRDEYLIVQGGALAGTGAHSYSKGNATGGSEEAAKFKKAV

SEQ ID NO: 16 - DNA, 43 bp, Artificial
  PCR Primer
cccaagcttaaggagatatacatgtccatcatcgtgataagcg

SEQ ID NO: 17 - DNA, 34 bp, Artificial
  PCR Primer
ataagaatgcggccgctcagaactgtgtcgggcg

SEQ ID NO: 18 - DNA, 7404 bp, Artificial
  Plasmid pET21a FDH D221G 7beta-HSDH
  CDS (5208)..(6422): FDH D221G
  CDS (6435)..(7226): 7beta-HSDH
tggcgaatgggacgcgccctgtagcggcgcattaagcgcggcgggtgtggtggttacgcgcagcgtgaccgctacacttgccagcgccctagcgcccgctcctttcgctttcttcccttcctttctcgccacgttcgccggctttccccgtcaagctctaaatcgggggctccctttagggttccgatttagtgctttacggcacctcgaccccaaaaaacttgattagggtgatggttcacgtagtgggccatcgccctgatagacggtttttcgccctttgacgttggagtccacgttctttaatagtggactcttgttccaaactggaacaacactcaaccctatctcggtctattcttttgatttataagggattttgccgatttcggcctattggttaaaaaatgagctgatttaacaaaaatttaacgcgaattttaacaaaatattaacgtttacaatttcaggtggcacttttcggggaaatgtgcgcggaacccctatttgtttatttttctaaatacattcaaatatgtatccgctcatgagacaataaccctgataaatgcttcaataatattgaaaaaggaagagtatgagtattcaacatttccgtgtcgcccttattcccttttttgcggcattttgccttcctgtttttgctcacccagaaacgctggtgaaagtaaaagatgctgaagatcagttgggtgcacgagtgggttacatcgaactggatctcaacagcggtaagatccttgagagttttcgccccgaagaacgttttccaatgatgagcacttttaaagttctgctatgtggcgcggtattatcccgtattgacgccgggcaagagcaactcggtcgccgcatacactattctcagaatgacttggttgagtactcaccagtcacagaaaagcatcttacggatggcatgacagtaagagaattatgcagtgctgccataaccatgagtgataacactgcggccaacttacttctgacaacgatcggaggaccgaaggagctaaccgcttttttgcacaacatgggggatcatgtaactcgccttgatcgttgggaaccggagctgaatgaagccataccaaacgacgagcgtgacaccacgatgcctgcagcaatggcaacaacgttgcgcaaactattaactggcgaactacttactctagcttcccggcaacaattaatagactggatggaggcggataaagttgcaggaccacttctgcgctcggcccttccggctggctggtttattgctgataaatctggagccggtgagcgtgggtctcgcggtatcattgcagcactggggccagatggtaagccctcccgtatcgtagttatctacacgacggggagtcaggcaactatggatgaacgaaatagacagatcgctgagataggtgcctcactgattaagcattggtaactgtcagaccaagtttactcatatatactttagattgatttaaaacttcatttttaatttaaaaggatctaggtgaagatcctttttgataatctcatgaccaaaatcccttaacgtgagttttcgttccactgagcgtcagaccccgtagaaaagatcaaaggatcttcttgagatcctttttttctgcgcgtaatctgctgcttgcaaacaaaaaaaccaccgctaccagcggtggtttgtttgccggatcaagagctaccaactctttttccgaaggtaactggcttcagcagagcgcagataccaaatactgtccttctagtgtagccgtagttaggccaccacttcaagaactctgtagcaccgcctacatacctcgctctgctaatcctgttaccagtggctgctgccagtggcgataagtcgtgtcttaccgggttggactcaagacgatagttaccggataaggcgcagcggtcgggctgaacggggggttcgtgcacacagcccagcttggagcgaacgacctacaccgaactgagatacctacagcgtgagctatgagaaagcgccacgcttcccgaagggagaaaggcggacaggtatccggtaagcggcagggtcggaacaggagagcgcacgagggagcttccagggggaaacgcctggtatctttatagtcctgtcgggtttcgccacctctgacttgagcgtcgatttttgtgatgctcgtcaggggggcggagcctatggaaaaacgccagcaacgcggcctttttacggttcctggccttttgctggccttttgctcacatgttctttcctgcgttatcccctgattctgtggataaccgtattaccgcctttgagtgagctgataccgctcgccgcagccgaacgaccgagcgcagcgagtcagtgagcgaggaagcggaagagcgcctgatgcggtattttctccttacgcatctgtgcggtatttcacaccgcatatatggtgcactctcagtacaatctgctctgatgccgcatagttaagccagtatacactccgctatcgctacgtgactgggtcatggctgcgccccgacacccgccaacacccgctgacgcgccctgacgggcttgtctgctcccggcatccgcttacagacaagctgtgaccgtctccgggagctgcatgtgtcagaggttttcaccgtcatcaccgaaacgcgcgaggcagctgcggtaaagctcatcagcgtggtcgtgaagcgattcacagatgtctgcctgttcatccgcgtccagctcgttgagtttctccagaagcgttaatgtctggcttctgataaagcgggccatgttaagggcggttttttcctgtttggtcactgatgcctccgtgtaagggggatttctgttcatgggggtaatgataccgatgaaacgagagaggatgctcacgatacgggttactgatgatgaacatgcccggttactggaacgttgtgagggtaaacaactggcggtatggatgcggcgggaccagagaaaaatcactcagggtcaatgccagcgcttcgttaatacagatgtaggtgttccacagggtagccagcagcatcctgcgatgcagatccggaacataatggtgcagggcgctgacttccgcgtttccagactttacgaaacacggaaaccgaagaccattcatgttgttgctcaggtcgcagacgttttgcagcagcagtcgcttcacgttcgctcgcgtatcggtgattcattctgctaaccagtaaggcaaccccgccagcctagccgggtcctcaacgacaggagcacgatcatgcgcacccgtggggccgccatgccggcgataatggcctgcttctcgccgaaacgtttggtggcgggaccagtgacgaaggcttgagcgagggcgtgcaagattccgaataccgcaagcgacaggccgatcatcgtcgcgctccagcgaaagcggtcctcgccgaaaatgacccagagcgctgccggcacctgtcctacgagttgcatgataaagaagacagtcataagtgcggcgacgatagtcatgccccgcgcccaccggaaggagctgactgggttgaaggctctcaagggcatcggtcgagatcccggtgcctaatgagtgagctaacttacattaattgcgttgcgctcactgcccgctttccagtcgggaaacctgtcgtgccagctgcattaatgaatcggccaacgcgcggggagaggcggtttgcgtattgggcgccagggtggtttttcttttcaccagtgagacgggcaacagctgattgcccttcaccgcctggccctgagagagttgcagcaagcggtccacgctggtttgccccagcaggcgaaaatcctgtttgatggtggttaacggcgggatataacatgagctgtcttcggtatcgtcgtatcccactaccgagatatccgcaccaacgcgcagcccggactcggtaatggcgcgcattgcgcccagcgccatctgatcgttggcaaccagcatcgcagtgggaacgatgccctcattcagcatttgcatggtttgttgaaaaccggacatggcactccagtcgccttcccgttccgctatcggctgaatttgattgcgagtgagatatttatgccagccagccagacgcagacgcgccgagacagaacttaatgggcccgctaacagcgcgatttgctggtgacccaatgcgaccagatgctccacgcccagtcgcgtaccgtcttcatgggagaaaataatactgttgatgggtgtctggtcagagacatcaagaaataacgccggaacattagtgcaggcagcttccacagcaatggcatcctggtcatccagcggatagttaatgatcagcccactgacgcgttgcgcgagaagattgtgcaccgccgctttacaggcttcgacgccgcttcgttctaccatcgacaccaccacgctggcacccagttgatcggcgcgagatttaatcgccgcgacaatttgcgacggcgcgtgcagggccagactggaggtggcaacgccaatcagcaacgactgtttgcccgccagttgttgtgccacgcggttgggaatgtaattcagctccgccatcgccgcttccactttttcccgcgttttcgcagaaacgtggctggcctggttcaccacgcgggaaacggtctgataagagacaccggcatactctgcgacatcgtataacgttactggtttcacattcaccaccctgaattgactctcttccgggcgctatcatgccataccgcgaaaggttttgcgccattcgatggtgtccgggatctcgacgctctcccttatgcgactcctgcattaggaagcagcccagtagtaggttgaggccgttgagcaccgccgccgcaaggaatggtgcatgcaaggagatggcgcccaacagtcccccggccacggggcctgccaccatacccacgccgaaacaagcgctcatgagcccgaagtggcgagcccgatcttccccatcggtgatgtcggcgatataggcgccagcaaccgcacctgtggcgccggtgatgccggccacgatgcgtccggcgtagaggatcgagatctcgatcccgcgaaattaatacgactcactataggggaattgtgagcggataacaattcccctctagaaataattttgtttaactttaagaaggagatatacatatgatggcaaaggtcctgtgcgttctttacgatgatccggtcgacggctacccgaagacctatgcccgcgacgatcttccgaagatcgaccactatccgggcggccagatcttgccgacgccgaaggccatcgacttcacgcccgggcagttgctcggctccgtctccggcgagctcggcctgcgcgaatatctcgaatccaacggccacaccctggtcgtgacctccgacaaggacggccccgactcggtgttcgagcgcgagctggtcgatgcggatgtcgtcatctcccagcccttctggccggcctatctgacgcccgagcgcatcgccaaggccaagaacctgaagctcgcgctcaccgccggcatcggttccgaccacgtcgatcttcagtcggctatcgaccgcaacgtcaccgtggcggaagtcacctactgcaactcgatcagcgtcgccgagcatgtggtgatgatgatcctgtcgctggtgcgcaactatctgccctcgcacgaatgggcgcggaagggcggctggaacatcgccgactgcgtctcccacgcctacgacctcgaggcgatgcatgtcggcaccgtggccgccggccgcatcggtctcgcggtgctgcgccgtctggcgccgttcgacgtgcacctgcactacaccggccgtcaccgcctgccggaatcggtcgagaaggagctcaacctcacctggcacgcgacccgcgaggacatgtatccggtttgcgacgtggtgacgctgaactgcccgctgcaccccgaaaccgagcacatgatcaatgacgagacgctgaagctgttcaagcgtggcgcctacatcgtcaacaccgcccgcggcaagctgtgcgaccgcgatgccgtggcacgtgcgctcgaatccggccggctggccggctatgccggcgacgtgtggttcccgcagccggcgccgaaggaccacccctggcggacgatgccctataacggcatgaccccgcacatctccggcaccacgctgaccgcgcaggcgcgttatgcggcgggcacccgcgagatcctggagtgcttcttcgagggccgtccgatccgcgacgaatacctcatcgtgcagggcggcgctcttgccggcaccggcgcgcattcctactcgaagggcaatgccaccggcggttcggaagaggccgccaagttcaagaaggcggctgagaattcgtgaaaggagatatacatgaacctgagggagaagtacggtgagtggggcctgatcctgggcgcgaccgagggcgtcggcaaggcgttctgcgagaagatcgccgccggcggcatgaacgtcgtcatggtcggccgtcgcgaggagaagctgaacgtgctcgcaggcgagatccgcgagacctacggcgtggagaccaaggtcgtgcgcgccgactttagccagcccggcgctgccgagaccgtcttcgccgcgaccgagggcctggacatgggcttcatgagctacgtggcctgcctgcacagcttcggtaagatccaggacaccccctgggagaagcacgaggccatgatcaacgtcaacgtcgtgaccttcctcaagtgcttccaccactacatgcggatctttgccgcccaggaccgcggcgccgtgatcaacgtctcgtcgatgaccggcatcagctccagcccctggaacggccagtacggcgcgggcaaggccttcatcctcaagatgaccgaggccgtggcctgcgagtgcgagggcaccggcgtcgacgtcgaggtcatcaccctcggcaccaccctaacccccagcctgctgtccaacctccccggcggcccgcagggcgaggccgtcatgaagatcgccctcacccccgaggagtgcgttgacgaggcctttgagaagctgggtaaggagctctccgtcatcgccggccagcgcaacaaggactccgtccacgactggaaggcaaaccacaccgaggacgagtacatccgctacatggggtcgttctaccgcgactagaagcttgcggccgcactcgagcaccaccaccaccaccactgagatccggctgctaacaaagcccgaaaggaagctgagttggctgctgccaccgctgagcaataactagcataaccccttggggcctctaaacgggtcttgaggggttttttgctgaaaggaggaactatatccggat

SEQ ID NO: 19 - protein, 404 aa, Artificial
  Synthetic Construct
MAKVLCVLYDDPVDGYPKTYARDDLPKIDHYPGGQILPTPKAIDFTPGQLLGSVSGELGLREYLESNGHTLVVTSDKDGPDSVFERELVDADVVISQPFWPAYLTPERIAKAKNLKLALTAGIGSDHVDLQSAIDRNVTVAEVTYCNSISVAEHVVMMILSLVRNYLPSHEWARKGGWNIADCVSHAYDLEAMHVGTVAAGRIGLAVLRRLAPFDVHLHYTGRHRLPESVEKELNLTWHATREDMYPVCDVVTLNCPLHPETEHMINDETLKLFKRGAYIVNTARGKLCDRDAVARALESGRLAGYAGDVWFPQPAPKDHPWRTMPYNGMTPHISGTTLTAQARYAAGTREILECFFEGRPIRDEYLIVQGGALAGTGAHSYSKGNATGGSEEAAKFKKAAENS

SEQ ID NO: 20 - protein, 263 aa, Artificial; identical to SEQ ID NO: 2
  Synthetic Construct

SEQ ID NO: 21 - DNA, 4302 bp, Artificial
  Plasmid pCOLA(mod) 3alpha-HSDH
  CDS (303)..(1076): 3alpha-HSDH
ggggaattgtgagcggataacaattcccctgtagaaataattttgtttaactttaataaggagatataccatgggcagcagccatcaccatcatcaccacagccaggatccgaattcgagctcggcgcgcctgcaggtcgacaagcttgcggccgcataatgcttaagtcgaacagaaagtaatcgtattgtacacggccgcataatcgaaattaatacgactcactataggggaattgtgagcggataacaattccccatcttagtatattagttaagtataagaaggagatatacatatgatgtccatcatcgtgataagcggctgcgccaccggcattggtgccgctacgcgcaaggtcctggaggcggccggtcaccagatcgtaggcatcgatatacgcgatgcggaagtgattgccgatctctcgacggccgaaggtcgaaagcaggcgattgccgatgtactggcgaagtgcagcaagggcatggacggcctggtgctgtgcgccggcctgggaccgcagaccaaggtgcttggcaatgtggtttcggtcaattattttggcgcgaccgagctgatggatgcctttttgccagcgctgaaaaaaggccatcagcccgcagccgtcgtcatctcgtccgtggcttccgcgcatctggcttttgacaagaacccactggcgctggcactggaagccggcgaggaagccaaggcccgcgccattgtcgaacatgcgggagagcagggcggaaatctggcctatgcgggcagcaagaatgctttgacggtggctgtgcgcaaacgcgccgccgcctggggcgaggctggcgtgcgcctgaacaccatcgcccccggtgcaaccgagactcccttgctgcaggcgggcctgcaggacccgcgctatggcgaatccattgccaagttcgttcctcccatgggccgccgtgccgagccgtccgagatggcgtcggtcatcgcctttttgatgagcccggccgcaagctatgtgcatggcgcgcagatcgtcattgatggcggcattgatgcggtgatgcgcccgacacagttctgagaattcgagctccgtcgacaagcttgcggccgcactcgagcaccaccaccaccaccactgagatccggctgctaacaaagcccgaaaggaagctgagttggctgctgccaccgctgagcaataactagcataaccccttggggcctctaaacgggtcttgaggggttttttgctgaaacctcaggcatttgagaagcacacggtcacactgcttccggtagtcaataaaccggtaaaccagcaatagacataagcggctatttaacgaccctgccctgaaccgacgacaagctgacgaccgggtctccgcaagtggcacttttcggggaaatgtgcgcggaacccctatttgtttatttttctaaatacattcaaatatgtatccgctcatgaattaattcttacgccccgccctgccactcatcgcagtactgttgtaattcattaagcattctgccgacatggaagccatcacagacggcatgatgaacctgaatcgccagcggcatcagcaccttgtcgccttgcgtataatatttgcctatggtgaaaacgggggcgaagaagttgtccatattggccacgtttaaatcaaaactggtgaaactcacccagggattggctgagacgaaaaacatattctcaataaaccctttagggaaataggccaggttttcaccgtaacacgccacatcttgcgaatatatgtgtagaaactgccggaaatcgtcgtggtattcactccagagcgatgaaaacgtttcagtttgctcatggaaaacggtgtaacaagggtgaacactatcccatatcaccagctcaccgtctttcattgccatacggaattccggatgagcattcatcaggcgggcaagaatgtgaataaaggccggataaaacttgtgcttatttttctttacggtctttaaaaaggccgtaatatccagctgaacggtctggttataggtacattgagcaactgactgaaatgcctcaaaatgttctttacgatgccattgggatatatcaacggtggtatatccagtgatttttttctccatactcttcctttttcaatattattgaagcatttatcagggttattgtctcatgagcggatacatatttgaatgtatttagaaaaataaacaaataggcatgctagcgcagaaacgtcctagaagatgccaggaggatacttagcagagagacaataaggccggagcgaagccgtttttccataggctccgcccccctgacgaacatcacgaaatctgacgctcaaatcagtggtggcgaaacccgacaggactataaagataccaggcgtttccccctgatggctccctcttgcgctctcctgttcccgtcctgcggcgtccgtgttgtggtggaggctttacccaaatcaccacgtcccgttccgtgtagacagttcgctccaagctgggctgtgtgcaagaaccccccgttcagcccgactgctgcgccttatccggtaactatcatcttgagtccaacccggaaagacacgacaaaacgccactggcagcagccattggtaactgagaattagtggatttagatatcgagagtcttgaagtggtggcctaacagaggctacactgaaaggacagtatttggtatctgcgctccactaaagccagttaccaggttaagcagttccccaactgacttaaccttcgatcaaaccgcctccccaggcggttttttcgtttacagagcaggagattacgacgatcgtaaaaggatctcaagaagatcctttacggattcccgacaccatcactctagatttcagtgcaatttatctcttcaaatgtagcacctgaagtcagccccatacgatataagttgtaattctcatgttagtcatgccccgcgcccaccggaaggagctgactgggttgaaggctctcaagggcatcggtcgagatcccggtgcctaatgagtgagctaacttacattaattgcgttgcgctcactgcccgctttccagtcgggaaacctgtcgtgccagctgcattaatgaatcggccaacgcgcggggagaggcggtttgcgtattgggcgccagggtggtttttcttttcaccagtgagacgggcaacagctgattgcccttcaccgcctggccctgagagagttgcagcaagcggtccacgctggtttgccccagcaggcgaaaatcctgtttgatggtggttaacggcgggatataacatgagctgtcttcggtatcgtcgtatcccactaccgagatgtccgcaccaacgcgcagcccggactcggtaatggcgcgcattgcgcccagcgccatctgatcgttggcaaccagcatcgcagtgggaacgatgccctcattcagcatttgcatggtttgttgaaaaccggacatggcactccagtcgccttcccgttccgctatcggctgaatttgattgcgagtgagatatttatgccagccagccagacgcagacgcgccgagacagaacttaatgggcccgctaacagcgcgatttgctggtgacccaatgcgaccagatgctccacgcccagtcgcgtaccgtcttcatgggagaaaataatactgttgatgggtgtctggtcagagacatcaagaaataacgccggaacattagtgcaggcagcttccacagcaatggcatcctggtcatccagcggatagttaatgatcagcccactgacgcgttgcgcgagaagattgtgcaccgccgctttacaggcttcgacgccgcttcgttctaccatcgacaccaccacgctggcacccagttgatcggcgcgagatttaatcgccgcgacaatttgcgacggcgcgtgcagggccagactggaggtggcaacgccaatcagcaacgactgtttgcccgccagttgttgtgccacgcggttgggaatgtaattcagctccgccatcgccgcttccactttttcccgcgttttcgcagaaacgtggctggcctggttcaccacgcgggaaacggtctgataagagacaccggcatactctgcgacatcgtataacgttactggtttcacattcaccaccctgaattgactctcttccgggcgctatcatgccataccgcgaaaggttttgcgccattcgatggtgtccgggatctcgacgctctcccttatgcgactcctgcattaggaaattaatacgactcactata

SEQ ID NO: 22 - protein, 257 aa, Artificial [sequence omitted]

SEQ ID NO: 23 - DNA, 29 bp, Artificial
  PCR Primer
cgatcatatggcaaaggtcctgtgcgttc

SEQ ID NO: 24 - DNA, 29 bp, Artificial
  PCR Primer
gctagaattctcagccgccttcttgaact

SEQ ID NO: 25 - DNA, 768 bp, Escherichia coli
  CDS (1)..(768)
gtgtttaattctgacaacctgagactcgacggaaaatgcgccatcatcacaggtgcgggtgcaggtattggtaaagaaatcgccattacattcgcgacagctggcgcatctgtggtggtcagtgatattaacgccgacgcagctaaccatgttgtagacgaaattcaacaactgggtggtcaggcatttgcctgccgttgtgatattacttccgaacaggaactctctgcactggcagactttgctatcagtaagctgggtaaagttgatattctggttaacaacgccggtggcggtggacctaaaccgtttgatatgccaatggcggattttcgccgtgcttatgaactgaatgtgttttcttttttccatctgtcacaacttgttgcgccagaaatggaaaaaaatggcggtggcgttattctgaccatcacttctatggcggcagaaaataaaaatataaacatgacttcctatgcatcatctaaagctgcggccagtcatctggtcagaaatatggcgtttgacctaggtgaaaaaaatattcgggtaaatggcattgcgccgggggcaatattaaccgatgccctgaaatccgttattacaccagaaattgaacaaaaaatgttacagcacacgccgatcagacgtctgggccaaccgcaagatattgctaacgcagcgctgttcctttgctcgcctgctgcgagctgggtaagcggacaaattctcaccgtctccggtggtggggtacaggagctcaattaa

SEQ ID NO: 26 - protein, 255 aa, Escherichia coli
VFNSDNLRLDGKCAIITGAGAGIGKEIAITFATAGASVVVSDINADAANHVVDEIQQLGGQAFACRCDITSEQELSALADFAISKLGKVDILVNNAGGGGPKPFDMPMADFRRAYELNVFSFFHLSQLVAPEMEKNGGGVILTITSMAAENKNINMTSYASSKAAASHLVRNMAFDLGEKNIRVNGIAPGAILTDALKSVITPEIEQKMLQHTPIRRLGQPQDIANAALFLCSPAASWVSGQILTVSGGGVQELN

SEQ ID NO: 27 - DNA, 53 bp, Artificial
  PCR Primer
aaaaaagcttataattatccttataggacgtcatggtgcgcccagatagggtg

SEQ ID NO: 28 - DNA, 60 bp, Artificial
  PCR Primer
cagattgtacaaatgtggtgataacagataagtcgtcatgtttaacttacctttctttgt

SEQ ID NO: 29 - DNA, 49 bp, Artificial
  PCR Primer
tgaacgcaagtttctaatttcggtttcctatcgatagaggaaagtgtct

SEQ ID NO: 30 - DNA, 29 bp, Artificial
  PCR Primer
cctgcactacaccggccgtcaccgcctgc

SEQ ID NO: 31 - DNA, 23 bp, Artificial
  PCR Primer
gctcgaattctcagaccgccttc

SEQ ID NO: 32 - DNA, 27 bp, Artificial
  PCR Primer
ttaattgagctcctgtaccccaccacc

SEQ ID NO: 33 - DNA, 30 bp, Artificial
  PCR Primer
gtgtttaattctgacaacctgagactcgac

SEQ ID NO: 34 - DNA, 1266 bp, Artificial
  FDH D221G Mutante mit His-Tag
  CDS (1)..(1266)
atggcaaaggtcctgtgcgttctttacgatgatccggtcgacggctacccgaagacctatgcccgcgacgatcttccgaagatcgaccactatccgggcggccagatcttgccgacgccgaaggccatcgacttcacgcccgggcagttgctcggctccgtctccggcgagctcggcctgcgcgaatatctcgaatccaacggccacaccctggtcgtgacctccgacaaggacggccccgactcggtgttcgagcgcgagctggtcgatgcggatgtcgtcatctcccagcccttctggccggcctatctgacgcccgagcgcatcgccaaggccaagaacctgaagctcgcgctcaccgccggcatcggttccgaccacgtcgatcttcagtcggctatcgaccgcaacgtcaccgtggcggaagtcacctactgcaactcgatcagcgtcgccgagcatgtggtgatgatgatcctgtcgctggtgcgcaactatctgccctcgcacgaatgggcgcggaagggcggctggaacatcgccgactgcgtctcccacgcctacgacctcgaggcgatgcatgtcggcaccgtggccgccggccgcatcggtctcgcggtgctgcgccgtctggcgccgttcgacgtgcacctgcactacaccggccgtcaccgcctgccggaatcggtcgagaaggagctcaacctcacctggcacgcgacccgcgaggacatgtatccggtttgcgacgtggtgacgctgaactgcccgctgcaccccgaaaccgagcacatgatcaatgacgagacgctgaagctgttcaagcgtggcgcctacatcgtcaacaccgcccgcggcaagctgtgcgaccgcgatgccgtggcacgtgcgctcgaatccggccggctggccggctatgccggcgacgtgtggttcccgcagccggcgccgaaggaccacccctggcggacgatgccctataacggcatgaccccgcacatctccggcaccacgctgaccgcgcaggcgcgttatgcggcgggcacccgcgagatcctggagtgcttcttcgagggccgtccgatccgcgacgaatacctcatcgtgcagggcggcgctcttgccggcaccggcgcgcattcctactcgaagggcaatgccaccggcggttcggaagaggccgccaagttcaagaaggcggctgagaattcgagctccgtcgacaagcttgcggccgcactcgagcaccaccaccaccaccactga

SEQ ID NO: 35 - protein, 421 aa, Artificial
  Synthetic Construct
MAKVLCVLYDDPVDGYPKTYARDDLPKIDHYPGGQILPTPKAIDFTPGQLLGSVSGELGLREYLESNGHTLVVTSDKDGPDSVFERELVDADVVISQPFWPAYLTPERIAKAKNLKLALTAGIGSDHVDLQSAIDRNVTVAEVTYCNSISVAEHVVMMILSLVRNYLPSHEWARKGGWNIADCVSHAYDLEAMHVGTVAAGRIGLAVLRRLAPFDVHLHYTGRHRLPESVEKELNLTWHATREDMYPVCDVVTLNCPLHPETEHMINDETLKLFKRGAYIVNTARGKLCDRDAVARALESGRLAGYAGDVWFPQPAPKDHPWRTMPYNGMTPHISGTTLTAQARYAAGTREILECFFEGRPIRDEYLIVQGGALAGTGAHSYSKGNATGGSEEAAKFKKAAENSSSVDKLAAALEHHHHHH

SEQ ID NO: 36 - protein, 401 aa, Mycobacterium vaccae
MAKVLCVLYDDPVDGYPKTYARDDLPKIDHYPGGQILPTPKAIDFTPGQLLGSVSGELGLREYLESNGHTLVVTSDKDGPDSVFERELVDADVVISQPFWPAYLTPERIAKAKNLKLALTAGIGSDHVDLQSAIDRNVTVAEVTYCNSISVAEHVVMMILSLVRNYLPSHEWARKGGWNIADCVSHAYDLEAMHVGTVAAGRIGLAVLRRLAPFDVHLHYTDRHRLPESVEKELNLTWHATREDMYPVCDVVTLNCPLHPETEHMINDETLKLFKRGAYIVNTARGKLCDRDAVARALESGRLAGYAGDVWFPQPAPKDHPWRTMPYNGMTPHISGTTLTAQARYAAGTREILECFFEGRPIRDEYLIVQGGALAGTGAHSYSKGNATGGSEEAAKFKKAV

SEQ ID NO: 37 - protein, 263 aa, artificial
  abgeleitet aus Collinsella aerofaciens (G39D)
MNLREKYGEWGLILGATEGVGKAFCEKIAAGGMNVVMVDRREEKLNVLAGEIRETYGVETKVVRADFSQPGAAETVFAATEGLDMGFMSYVACLHSFGKIQDTPWEKHEAMINVNVVTFLKCFHHYMRIFAAQDRGAVINVSSMTGISSSPWNGQYGAGKAFILKMTEAVACECEGTGVDVEVITLGTTLTPSLLSNLPGGPQGEAVMKIALTPEECVDEAFEKLGKELSVIAGQRNKDSVHDWKANHTEDEYIRYMGSFYRD

SEQ ID NO: 38 - protein, 263 aa, artificial
  abgeleitet aus Collinsella aerofaciens (G39D R40L)
MNLREKYGEWGLILGATEGVGKAFCEKIAAGGMNVVMVDLREEKLNVLAGEIRETYGVETKVVRADFSQPGAAETVFAATEGLDMGFMSYVACLHSFGKIQDTPWEKHEAMINVNVVTFLKCFHHYMRIFAAQDRGAVINVSSMTGISSSPWNGQYGAGKAFILKMTEAVACECEGTGVDVEVITLGTTLTPSLLSNLPGGPQGEAVMKIALTPEECVDEAFEKLGKELSVIAGQRNKDSVHDWKANHTEDEYIRYMGSFYRD

SEQ ID NO: 39 - protein, 263 aa, artificial
  abegleitet aus Collinsella aerofaciens (G39D R40I)
MNLREKYGEWGLILGATEGVGKAFCEKIAAGGMNVVMVDIREEKLNVLAGEIRETYGVETKVVRADFSQPGAAETVFAATEGLDMGFMSYVACLHSFGKIQDTPWEKHEAMINVNVVTFLKCFHHYMRIFAAQDRGAVINVSSMTGISSSPWNGQYGAGKAFILKMTEAVACECEGTGVDVEVITLGTTLTPSLLSNLPGGPQGEAVMKIALTPEECVDEAFEKLGKELSVIAGQRNKDSVHDWKANHTEDEYIRYMGSFYRD

SEQ ID NO: 40 - protein, 263 aa, artificial
  abgeleitet aus Collinsella aerofaciens
MNLREKYGEWGLILGATEGVGKAFCEKIAAGGMNVVMVDVREEKLNVLAGEIRETYGVETKVVRADFSQPGAAETVFAATEGLDMGFMSYVACLHSFGKIQDTPWEKHEAMINVNVVTFLKCFHHYMRIFAAQDRGAVINVSSMTGISSSPWNGQYGAGKAFILKMTEAVACECEGTGVDVEVITLGTTLTPSLLSNLPGGPQGEAVMKIALTPEECVDEAFEKLGKELSVIAGQRNKDSVHDWKANHTEDEYIRYMGSFYRD

SEQ ID NO: 41 - DNA, 26 bp, artificial
  PCR Primer
cgtcgtcatggtcgaccgtcgcgagg

SEQ ID NO: 42 - DNA, 26 bp, artificial
  PCR Primer
cctcgcgacggtcgaccatgacgacg

SEQ ID NO: 43 - DNA, 26 bp, artificial
  PCR Primer
cgtcgtcatggtcgacctgcgcgagg

SEQ ID NO: 44 - DNA, 31 bp, artificial
  PCR Primer
ccgccgcatccataccgccagttgtttaccc

SEQ ID NO: 45 - DNA, 26 bp, artificial
  PCR Primer
cgtcgtcatggtcgacattcgcgagg

SEQ ID NO: 46 - DNA, 26 bp, artificial
  PCR Primer
cgtcgtcatggtcgacgttcgcgagg

SEQ ID NO: 47 - DNA, 786 bp, Bacillus subtilis
atgtatccggatttaaaaggaaaagtcgtcgctattacaggagctgcttcagggctcggaaaggcgatggccattcgcttcggcaaggagcaggcaaaagtggttatcaactattatagtaataaacaagatccgaacgaggtaaaagaagaggtcatcaaggcgggcggtgaagctgttgtcgtccaaggagatgtcacgaaagaggaagatgtaaaaaatatcgtgcaaacggcaattaaggagttcggcacactcgatattatgattaataatgccggtcttgaaaatcctgtgccatctcacgaaatgccgctcaaggattgggataaagtcatcggcacgaacttaacgggtgcctttttaggaagccgtgaagcgattaaatatttcgtagaaaacgatatcaagggaaatgtcattaacatgtccagtgtgcacgaagtgattccttggccgttatttgtccactatgcggcaagtaaaggcgggataaagctgatgacagaaacattagcgttggaatacgcgccgaagggcattcgcgtcaataatattgggccaggtgcgatcaacacgccaatcaatgctgaaaaattcgctgaccctaaacagaaagctgatgtagaaagcatgattccaatgggatatatcggcgaaccggaggagatcgccgcagtagcagcctggcttgcttcgaaggaagccagctacgtcacaggcatcacgttattcgcggacggcggtatgacacaatatccttcattccaggcaggccgcggttaa

SEQ ID NO: 48 - protein, 261 aa, Bacillus subtilis
MYPDLKGKVVAITGAASGLGKAMAIRFGKEQAKVVINYYSNKQDPNEVKEEVIKAGGEAVVVQGDVTKEEDVKNIVQTAIKEFGTLDIMINNAGLENPVPSHEMPLKDWDKVIGTNLTGAFLGSREAIKYFVENDIKGNVINMSSVHEVIPWPLFVHYAASKGGIKLMTETLALEYAPKGIRVNNIGPGAINTPINAEKFADPKQKADVESMIPMGYIGEPEEIAAVAAWLASKEASYVTGITLFADGGMTQYPSFQAGRG

SEQ ID NO: 49 - DNA, 7404 bp, artificial
  Vektor pFr7(D)
atccggatatagttcctcctttcagcaaaaaacccctcaagacccgtttagaggccccaaggggttatgctagttattgctcagcggtggcagcagccaactcagcttcctttcgggctttgttagcagccggatctcagtggtggtggtggtggtgctcgagtgcggccgcaagcttctagtcgcggtagaacgaccccatgtagcggatgtactcgtcctcggtgtggtttgccttccagtcgtggacggagtccttgttgcgctggccggcgatgacggagagctccttacccagcttctcaaaggcctcgtcaacgcactcctcgggggtgagggcgatcttcatgacggcctcgccctgcgggccgccggggaggttggacagcaggctgggggttagggtggtgccgagggtgatgacctcgacgtcgacgccggtgccctcgcactcgcaggccacggcctcggtcatcttgaggatgaaggccttgcccgcgccgtactggccgttccaggggctggagctgatgccggtcatcgacgagacgttgatcacggcgccgcggtcctgggcggcaaagatccgcatgtagtggtggaagcacttgaggaaggtcacgacgttgacgttgatcatggcctcgtgcttctcccagggggtgtcctggatcttaccgaagctgtgcaggcaggccacgtagctcatgaagcccatgtccaggccctcggtcgcggcgaagacggtctcggcagcgccgggctggctaaagtcggcgcgcacgaccttggtctccacgccgtaggtctcgcggatctcgcctgcgagcacgttcagcttctcctcgcgacggtcgaccatgacgacgttcatgccgccggcggcgatcttctcgcagaacgccttgccgacgccctcggtcgcgcccaggatcaggccccactcaccgtacttctccctcaggttcatgtatatctcctttcacgaattctcagccgccttcttgaacttggcggcctcttccgaaccgccggtggcattgcccttcgagtaggaatgcgcgccggtgccggcaagagcgccgccctgcacgatgaggtattcgtcgcggatcggacggccctcgaagaagcactccaggatctcgcgggtgcccgccgcataacgcgcctgcgcggtcagcgtggtgccggagatgtgcggggtcatgccgttatagggcatcgtccgccaggggtggtccttcggcgccggctgcgggaaccacacgtcgccggcatagccggccagccggccggattcgagcgcacgtgccacggcatcgcggtcgcacagcttgccgcgggcggtgttgacgatgtaggcgccacgcttgaacagcttcagcgtctcgtcattgatcatgtgctcggtttcggggtgcagcgggcagttcagcgtcaccacgtcgcaaaccggatacatgtcctcgcgggtcgcgtgccaggtgaggttgagctccttctcgaccgattccggcaggcggtgacggccggtgtagtgcaggtgcacgtcgaacggcgccagacggcgcagcaccgcgagaccgatgcggccggcggccacggtgccgacatgcatcgcctcgaggtcgtaggcgtgggagacgcagtcggcgatgttccagccgcccttccgcgcccattcgtgcgagggcagatagttgcgcaccagcgacaggatcatcatcaccacatgctcggcgacgctgatcgagttgcagtaggtgacttccgccacggtgacgttgcggtcgatagccgactgaagatcgacgtggtcggaaccgatgccggcggtgagcgcgagcttcaggttcttggccttggcgatgcgctcgggcgtcagataggccggccagaagggctgggagatgacgacatccgcatcgaccagctcgcgctcgaacaccgagtcggggccgtccttgtcggaggtcacgaccagggtgtggccgttggattcgagatattcgcgcaggccgagctcgccggagacggagccgagcaactgcccgggcgtgaagtcgatggccttcggcgtcggcaagatctggccgcccggatagtggtcgatcttcggaagatcgtcgcgggcataggtcttcgggtagccgtcgaccggatcatcgtaaagaacgcacaggacctttgccatcatatgtatatctccttcttaaagttaaacaaaattatttctagaggggaattgttatccgctcacaattcccctatagtgagtcgtattaatttcgcgggatcgagatctcgatcctctacgccggacgcatcgtggccggcatcaccggcgccacaggtgcggttgctggcgcctatatcgccgacatcaccgatggggaagatcgggctcgccacttcgggctcatgagcgcttgtttcggcgtgggtatggtggcaggccccgtggccgggggactgttgggcgccatctccttgcatgcaccattccttgcggcggcggtgctcaacggcctcaacctactactgggctgcttcctaatgcaggagtcgcataagggagagcgtcgagatcccggacaccatcgaatggcgcaaaacctttcgcggtatggcatgatagcgcccggaagagagtcaattcagggtggtgaatgtgaaaccagtaacgttatacgatgtcgcagagtatgccggtgtctcttatcagaccgtttcccgcgtggtgaaccaggccagccacgtttctgcgaaaacgcgggaaaaagtggaagcggcgatggcggagctgaattacattcccaaccgcgtggcacaacaactggcgggcaaacagtcgttgctgattggcgttgccacctccagtctggccctgcacgcgccgtcgcaaattgtcgcggcgattaaatctcgcgccgatcaactgggtgccagcgtggtggtgtcgatggtagaacgaagcggcgtcgaagcctgtaaagcggcggtgcacaatcttctcgcgcaacgcgtcagtgggctgatcattaactatccgctggatgaccaggatgccattgctgtggaagctgcctgcactaatgttccggcgttatttcttgatgtctctgaccagacacccatcaacagtattattttctcccatgaagacggtacgcgactgggcgtggagcatctggtcgcattgggtcaccagcaaatcgcgctgttagcgggcccattaagttctgtctcggcgcgtctgcgtctggctggctggcataaatatctcactcgcaatcaaattcagccgatagcggaacgggaaggcgactggagtgccatgtccggttttcaacaaaccatgcaaatgctgaatgagggcatcgttcccactgcgatgctggttgccaacgatcagatggcgctgggcgcaatgcgcgccattaccgagtccgggctgcgcgttggtgcggatatctcggtagtgggatacgacgataccgaagacagctcatgttatatcccgccgttaaccaccatcaaacaggattttcgcctgctggggcaaaccagcgtggaccgcttgctgcaactctctcagggccaggcggtgaagggcaatcagctgttgcccgtctcactggtgaaaagaaaaaccaccctggcgcccaatacgcaaaccgcctctccccgcgcgttggccgattcattaatgcagctggcacgacaggtttcccgactggaaagcgggcagtgagcgcaacgcaattaatgtaagttagctcactcattaggcaccgggatctcgaccgatgcccttgagagccttcaacccagtcagctccttccggtgggcgcggggcatgactatcgtcgccgcacttatgactgtcttctttatcatgcaactcgtaggacaggtgccggcagcgctctgggtcattttcggcgaggaccgctttcgctggagcgcgacgatgatcggcctgtcgcttgcggtattcggaatcttgcacgccctcgctcaagccttcgtcactggtcccgccaccaaacgtttcggcgagaagcaggccattatcgccggcatggcggccccacgggtgcgcatgatcgtgctcctgtcgttgaggacccggctaggctggcggggttgccttactggttagcagaatgaatcaccgatacgcgagcgaacgtgaagcgactgctgctgcaaaacgtctgcgacctgagcaacaacatgaatggtcttcggtttccgtgtttcgtaaagtctggaaacgcggaagtcagcgccctgcaccattatgttccggatctgcatcgcaggatgctgctggctaccctgtggaacacctacatctgtattaacgaagcgctggcattgaccctgagtgatttttctctggtcccgccgcatccataccgccagttgtttaccctcacaacgttccagtaaccgggcatgttcatcatcagtaacccgtatcgtgagcatcctctctcgtttcatcggtatcattacccccatgaacagaaatcccccttacacggaggcatcagtgaccaaacaggaaaaaaccgcccttaacatggcccgctttatcagaagccagacattaacgcttctggagaaactcaacgagctggacgcggatgaacaggcagacatctgtgaatcgcttcacgaccacgctgatgagctttaccgcagctgcctcgcgcgtttcggtgatgacggtgaaaacctctgacacatgcagctcccggagacggtcacagcttgtctgtaagcggatgccgggagcagacaagcccgtcagggcgcgtcagcgggtgttggcgggtgtcggggcgcagccatgacccagtcacgtagcgatagcggagtgtatactggcttaactatgcggcatcagagcagattgtactgagagtgcaccatatatgcggtgtgaaataccgcacagatgcgtaaggagaaaataccgcatcaggcgctcttccgcttcctcgctcactgactcgctgcgctcggtcgttcggctgcggcgagcggtatcagctcactcaaaggcggtaatacggttatccacagaatcaggggataacgcaggaaagaacatgtgagcaaaaggccagcaaaaggccaggaaccgtaaaaaggccgcgttgctggcgtttttccataggctccgcccccctgacgagcatcacaaaaatcgacgctcaagtcagaggtggcgaaacccgacaggactataaagataccaggcgtttccccctggaagctccctcgtgcgctctcctgttccgaccctgccgcttaccggatacctgtccgcctttctcccttcgggaagcgtggcgctttctcatagctcacgctgtaggtatctcagttcggtgtaggtcgttcgctccaagctgggctgtgtgcacgaaccccccgttcagcccgaccgctgcgccttatccggtaactatcgtcttgagtccaacccggtaagacacgacttatcgccactggcagcagccactggtaacaggattagcagagcgaggtatgtaggcggtgctacagagttcttgaagtggtggcctaactacggctacactagaaggacagtatttggtatctgcgctctgctgaagccagttaccttcggaaaaagagttggtagctcttgatccggcaaacaaaccaccgctggtagcggtggtttttttgtttgcaagcagcagattacgcgcagaaaaaaaggatctcaagaagatcctttgatcttttctacggggtctgacgctcagtggaacgaaaactcacgttaagggattttggtcatgagattatcaaaaaggatcttcacctagatccttttaaattaaaaatgaagttttaaatcaatctaaagtatatatgagtaaacttggtctgacagttaccaatgcttaatcagtgaggcacctatctcagcgatctgtctatttcgttcatccatagttgcctgactccccgtcgtgtagataactacgatacgggagggcttaccatctggccccagtgctgcaatgataccgcgagacccacgctcaccggctccagatttatcagcaataaaccagccagccggaagggccgagcgcagaagtggtcctgcaactttatccgcctccatccagtctattaattgttgccgggaagctagagtaagtagttcgccagttaatagtttgcgcaacgttgttgccattgctgcaggcatcgtggtgtcacgctcgtcgtttggtatggcttcattcagctccggttcccaacgatcaaggcgagttacatgatcccccatgttgtgcaaaaaagcggttagctccttcggtcctccgatcgttgtcagaagtaagttggccgcagtgttatcactcatggttatggcagcactgcataattctcttactgtcatgccatccgtaagatgcttttctgtgactggtgagtactcaaccaagtcattctgagaatagtgtatgcggcgaccgagttgctcttgcccggcgtcaatacgggataataccgcgccacatagcagaactttaaaagtgctcatcattggaaaacgttcttcggggcgaaaactctcaaggatcttaccgctgttgagatccagttcgatgtaacccactcgtgcacccaactgatcttcagcatcttttactttcaccagcgtttctgggtgagcaaaaacaggaaggcaaaatgccgcaaaaaagggaataagggcgacacggaaatgttgaatactcatactcttcctttttcaatattattgaagcatttatcagggttattgtctcatgagcggatacatatttgaatgtatttagaaaaataaacaaataggggttccgcgcacatttccccgaaaagtgccacctgaaattgtaaacgttaatattttgttaaaattcgcgttaaatttttgttaaatcagctcattttttaaccaataggccgaaatcggcaaaatcccttataaatcaaaagaatagaccgagatagggttgagtgttgttccagtttggaacaagagtccactattaaagaacgtggactccaacgtcaaagggcgaaaaaccgtctatcagggcgatggcccactacgtgaaccatcaccctaatcaagttttttggggtcgaggtgccgtaaagcactaaatcggaaccctaaagggagcccccgatttagagcttgacggggaaagccggcgaacgtggcgagaaaggaagggaagaaagcgaaaggagcgggcgctagggcgctggcaagtgtagcggtcacgctgcgcgtaaccaccacacccgccgcgcttaatgcgccgctacagggcgcgtcccattcgcca

SEQ ID NO: 50 - DNA, 7404 bp, artificial
  Vektor pFr7(DL)
atccggatatagttcctcctttcagcaaaaaacccctcaagacccgtttagaggccccaaggggttatgctagttattgctcagcggtggcagcagccaactcagcttcctttcgggctttgttagcagccggatctcagtggtggtggtggtggtgctcgagtgcggccgcaagcttctagtcgcggtagaacgaccccatgtagcggatgtactcgtcctcggtgtggtttgccttccagtcgtggacggagtccttgttgcgctggccggcgatgacggagagctccttacccagcttctcaaaggcctcgtcaacgcactcctcgggggtgagggcgatcttcatgacggcctcgccctgcgggccgccggggaggttggacagcaggctgggggttagggtggtgccgagggtgatgacctcgacgtcgacgccggtgccctcgcactcgcaggccacggcctcggtcatcttgaggatgaaggccttgcccgcgccgtactggccgttccaggggctggagctgatgccggtcatcgacgagacgttgatcacggcgccgcggtcctgggcggcaaagatccgcatgtagtggtggaagcacttgaggaaggtcacgacgttgacgttgatcatggcctcgtgcttctcccagggggtgtcctggatcttaccgaagctgtgcaggcaggccacgtagctcatgaagcccatgtccaggccctcggtcgcggcgaagacggtctcggcagcgccgggctggctaaagtcggcgcgcacgaccttggtctccacgccgtaggtctcgcggatctcgcctgcgagcacgttcagcttctcctcgcgcaggtcgaccatgacgacgttcatgccgccggcggcgatcttctcgcagaacgccttgccgacgccctcggtcgcgcccaggatcaggccccactcaccgtacttctccctcaggttcatgtatatctcctttcacgaattctcagccgccttcttgaacttggcggcctcttccgaaccgccggtggcattgcccttcgagtaggaatgcgcgccggtgccggcaagagcgccgccctgcacgatgaggtattcgtcgcggatcggacggccctcgaagaagcactccaggatctcgcgggtgcccgccgcataacgcgcctgcgcggtcagcgtggtgccggagatgtgcggggtcatgccgttatagggcatcgtccgccaggggtggtccttcggcgccggctgcgggaaccacacgtcgccggcatagccggccagccggccggattcgagcgcacgtgccacggcatcgcggtcgcacagcttgccgcgggcggtgttgacgatgtaggcgccacgcttgaacagcttcagcgtctcgtcattgatcatgtgctcggtttcggggtgcagcgggcagttcagcgtcaccacgtcgcaaaccggatacatgtcctcgcgggtcgcgtgccaggtgaggttgagctccttctcgaccgattccggcaggcggtgacggccggtgtagtgcaggtgcacgtcgaacggcgccagacggcgcagcaccgcgagaccgatgcggccggcggccacggtgccgacatgcatcgcctcgaggtcgtaggcgtgggagacgcagtcggcgatgttccagccgcccttccgcgcccattcgtgcgagggcagatagttgcgcaccagcgacaggatcatcatcaccacatgctcggcgacgctgatcgagttgcagtaggtgacttccgccacggtgacgttgcggtcgatagccgactgaagatcgacgtggtcggaaccgatgccggcggtgagcgcgagcttcaggttcttggccttggcgatgcgctcgggcgtcagataggccggccagaagggctgggagatgacgacatccgcatcgaccagctcgcgctcgaacaccgagtcggggccgtccttgtcggaggtcacgaccagggtgtggccgttggattcgagatattcgcgcaggccgagctcgccggagacggagccgagcaactgcccgggcgtgaagtcgatggccttcggcgtcggcaagatctggccgcccggatagtggtcgatcttcggaagatcgtcgcgggcataggtcttcgggtagccgtcgaccggatcatcgtaaagaacgcacaggacctttgccatcatatgtatatctccttcttaaagttaaacaaaattatttctagaggggaattgttatccgctcacaattcccctatagtgagtcgtattaatttcgcgggatcgagatctcgatcctctacgccggacgcatcgtggccggcatcaccggcgccacaggtgcggttgctggcgcctatatcgccgacatcaccgatggggaagatcgggctcgccacttcgggctcatgagcgcttgtttcggcgtgggtatggtggcaggccccgtggccgggggactgttgggcgccatctccttgcatgcaccattccttgcggcggcggtgctcaacggcctcaacctactactgggctgcttcctaatgcaggagtcgcataagggagagcgtcgagatcccggacaccatcgaatggcgcaaaacctttcgcggtatggcatgatagcgcccggaagagagtcaattcagggtggtgaatgtgaaaccagtaacgttatacgatgtcgcagagtatgccggtgtctcttatcagaccgtttcccgcgtggtgaaccaggccagccacgtttctgcgaaaacgcgggaaaaagtggaagcggcgatggcggagctgaattacattcccaaccgcgtggcacaacaactggcgggcaaacagtcgttgctgattggcgttgccacctccagtctggccctgcacgcgccgtcgcaaattgtcgcggcgattaaatctcgcgccgatcaactgggtgccagcgtggtggtgtcgatggtagaacgaagcggcgtcgaagcctgtaaagcggcggtgcacaatcttctcgcgcaacgcgtcagtgggctgatcattaactatccgctggatgaccaggatgccattgctgtggaagctgcctgcactaatgttccggcgttatttcttgatgtctctgaccagacacccatcaacagtattattttctcccatgaagacggtacgcgactgggcgtggagcatctggtcgcattgggtcaccagcaaatcgcgctgttagcgggcccattaagttctgtctcggcgcgtctgcgtctggctggctggcataaatatctcactcgcaatcaaattcagccgatagcggaacgggaaggcgactggagtgccatgtccggttttcaacaaaccatgcaaatgctgaatgagggcatcgttcccactgcgatgctggttgccaacgatcagatggcgctgggcgcaatgcgcgccattaccgagtccgggctgcgcgttggtgcggatatctcggtagtgggatacgacgataccgaagacagctcatgttatatcccgccgttaaccaccatcaaacaggattttcgcctgctggggcaaaccagcgtggaccgcttgctgcaactctctcagggccaggcggtgaagggcaatcagctgttgcccgtctcactggtgaaaagaaaaaccaccctggcgcccaatacgcaaaccgcctctccccgcgcgttggccgattcattaatgcagctggcacgacaggtttcccgactggaaagcgggcagtgagcgcaacgcaattaatgtaagttagctcactcattaggcaccgggatctcgaccgatgcccttgagagccttcaacccagtcagctccttccggtgggcgcggggcatgactatcgtcgccgcacttatgactgtcttctttatcatgcaactcgtaggacaggtgccggcagcgctctgggtcattttcggcgaggaccgctttcgctggagcgcgacgatgatcggcctgtcgcttgcggtattcggaatcttgcacgccctcgctcaagccttcgtcactggtcccgccaccaaacgtttcggcgagaagcaggccattatcgccggcatggcggccccacgggtgcgcatgatcgtgctcctgtcgttgaggacccggctaggctggcggggttgccttactggttagcagaatgaatcaccgatacgcgagcgaacgtgaagcgactgctgctgcaaaacgtctgcgacctgagcaacaacatgaatggtcttcggtttccgtgtttcgtaaagtctggaaacgcggaagtcagcgccctgcaccattatgttccggatctgcatcgcaggatgctgctggctaccctgtggaacacctacatctgtattaacgaagcgctggcattgaccctgagtgatttttctctggtcccgccgcatccataccgccagttgtttaccctcacaacgttccagtaaccgggcatgttcatcatcagtaacccgtatcgtgagcatcctctctcgtttcatcggtatcattacccccatgaacagaaatcccccttacacggaggcatcagtgaccaaacaggaaaaaaccgcccttaacatggcccgctttatcagaagccagacattaacgcttctggagaaactcaacgagctggacgcggatgaacaggcagacatctgtgaatcgcttcacgaccacgctgatgagctttaccgcagctgcctcgcgcgtttcggtgatgacggtgaaaacctctgacacatgcagctcccggagacggtcacagcttgtctgtaagcggatgccgggagcagacaagcccgtcagggcgcgtcagcgggtgttggcgggtgtcggggcgcagccatgacccagtcacgtagcgatagcggagtgtatactggcttaactatgcggcatcagagcagattgtactgagagtgcaccatatatgcggtgtgaaataccgcacagatgcgtaaggagaaaataccgcatcaggcgctcttccgcttcctcgctcactgactcgctgcgctcggtcgttcggctgcggcgagcggtatcagctcactcaaaggcggtaatacggttatccacagaatcaggggataacgcaggaaagaacatgtgagcaaaaggccagcaaaaggccaggaaccgtaaaaaggccgcgttgctggcgtttttccataggctccgcccccctgacgagcatcacaaaaatcgacgctcaagtcagaggtggcgaaacccgacaggactataaagataccaggcgtttccccctggaagctccctcgtgcgctctcctgttccgaccctgccgcttaccggatacctgtccgcctttctcccttcgggaagcgtggcgctttctcatagctcacgctgtaggtatctcagttcggtgtaggtcgttcgctccaagctgggctgtgtgcacgaaccccccgttcagcccgaccgctgcgccttatccggtaactatcgtcttgagtccaacccggtaagacacgacttatcgccactggcagcagccactggtaacaggattagcagagcgaggtatgtaggcggtgctacagagttcttgaagtggtggcctaactacggctacactagaaggacagtatttggtatctgcgctctgctgaagccagttaccttcggaaaaagagttggtagctcttgatccggcaaacaaaccaccgctggtagcggtggtttttttgtttgcaagcagcagattacgcgcagaaaaaaaggatctcaagaagatcctttgatcttttctacggggtctgacgctcagtggaacgaaaactcacgttaagggattttggtcatgagattatcaaaaaggatcttcacctagatccttttaaattaaaaatgaagttttaaatcaatctaaagtatatatgagtaaacttggtctgacagttaccaatgcttaatcagtgaggcacctatctcagcgatctgtctatttcgttcatccatagttgcctgactccccgtcgtgtagataactacgatacgggagggcttaccatctggccccagtgctgcaatgataccgcgagacccacgctcaccggctccagatttatcagcaataaaccagccagccggaagggccgagcgcagaagtggtcctgcaactttatccgcctccatccagtctattaattgttgccgggaagctagagtaagtagttcgccagttaatagtttgcgcaacgttgttgccattgctgcaggcatcgtggtgtcacgctcgtcgtttggtatggcttcattcagctccggttcccaacgatcaaggcgagttacatgatcccccatgttgtgcaaaaaagcggttagctccttcggtcctccgatcgttgtcagaagtaagttggccgcagtgttatcactcatggttatggcagcactgcataattctcttactgtcatgccatccgtaagatgcttttctgtgactggtgagtactcaaccaagtcattctgagaatagtgtatgcggcgaccgagttgctcttgcccggcgtcaatacgggataataccgcgccacatagcagaactttaaaagtgctcatcattggaaaacgttcttcggggcgaaaactctcaaggatcttaccgctgttgagatccagttcgatgtaacccactcgtgcacccaactgatcttcagcatcttttactttcaccagcgtttctgggtgagcaaaaacaggaaggcaaaatgccgcaaaaaagggaataagggcgacacggaaatgttgaatactcatactcttcctttttcaatattattgaagcatttatcagggttattgtctcatgagcggatacatatttgaatgtatttagaaaaataaacaaataggggttccgcgcacatttccccgaaaagtgccacctgaaattgtaaacgttaatattttgttaaaattcgcgttaaatttttgttaaatcagctcattttttaaccaataggccgaaatcggcaaaatcccttataaatcaaaagaatagaccgagatagggttgagtgttgttccagtttggaacaagagtccactattaaagaacgtggactccaacgtcaaagggcgaaaaaccgtctatcagggcgatggcccactacgtgaaccatcaccctaatcaagttttttggggtcgaggtgccgtaaagcactaaatcggaaccctaaagggagcccccgatttagagcttgacggggaaagccggcgaacgtggcgagaaaggaagggaagaaagcgaaaggagcgggcgctagggcgctggcaagtgtagcggtcacgctgcgcgtaaccaccacacccgccgcgcttaatgcgccgctacagggcgcgtcccattcgcca

SEQ ID NO: 51 - DNA, 7404 bp, artificial
  Vektor pFr7(DI)
atccggatatagttcctcctttcagcaaaaaacccctcaagacccgtttagaggccccaaggggttatgctagttattgctcagcggtggcagcagccaactcagcttcctttcgggctttgttagcagccggatctcagtggtggtggtggtggtgctcgagtgcggccgcaagcttctagtcgcggtagaacgaccccatgtagcggatgtactcgtcctcggtgtggtttgccttccagtcgtggacggagtccttgttgcgctggccggcgatgacggagagctccttacccagcttctcaaaggcctcgtcaacgcactcctcgggggtgagggcgatcttcatgacggcctcgccctgcgggccgccggggaggttggacagcaggctgggggttagggtggtgccgagggtgatgacctcgacgtcgacgccggtgccctcgcactcgcaggccacggcctcggtcatcttgaggatgaaggccttgcccgcgccgtactggccgttccaggggctggagctgatgccggtcatcgacgagacgttgatcacggcgccgcggtcctgggcggcaaagatccgcatgtagtggtggaagcacttgaggaaggtcacgacgttgacgttgatcatggcctcgtgcttctcccagggggtgtcctggatcttaccgaagctgtgcaggcaggccacgtagctcatgaagcccatgtccaggccctcggtcgcggcgaagacggtctcggcagcgccgggctggctaaagtcggcgcgcacgaccttggtctccacgccgtaggtctcgcggatctcgcctgcgagcacgttcagcttctcctcgcgaatgtcgaccatgacgacgttcatgccgccggcggcgatcttctcgcagaacgccttgccgacgccctcggtcgcgcccaggatcaggccccactcaccgtacttctccctcaggttcatgtatatctcctttcacgaattctcagccgccttcttgaacttggcggcctcttccgaaccgccggtggcattgcccttcgagtaggaatgcgcgccggtgccggcaagagcgccgccctgcacgatgaggtattcgtcgcggatcggacggccctcgaagaagcactccaggatctcgcgggtgcccgccgcataacgcgcctgcgcggtcagcgtggtgccggagatgtgcggggtcatgccgttatagggcatcgtccgccaggggtggtccttcggcgccggctgcgggaaccacacgtcgccggcatagccggccagccggccggattcgagcgcacgtgccacggcatcgcggtcgcacagcttgccgcgggcggtgttgacgatgtaggcgccacgcttgaacagcttcagcgtctcgtcattgatcatgtgctcggtttcggggtgcagcgggcagttcagcgtcaccacgtcgcaaaccggatacatgtcctcgcgggtcgcgtgccaggtgaggttgagctccttctcgaccgattccggcaggcggtgacggccggtgtagtgcaggtgcacgtcgaacggcgccagacggcgcagcaccgcgagaccgatgcggccggcggccacggtgccgacatgcatcgcctcgaggtcgtaggcgtgggagacgcagtcggcgatgttccagccgcccttccgcgcccattcgtgcgagggcagatagttgcgcaccagcgacaggatcatcatcaccacatgctcggcgacgctgatcgagttgcagtaggtgacttccgccacggtgacgttgcggtcgatagccgactgaagatcgacgtggtcggaaccgatgccggcggtgagcgcgagcttcaggttcttggccttggcgatgcgctcgggcgtcagataggccggccagaagggctgggagatgacgacatccgcatcgaccagctcgcgctcgaacaccgagtcggggccgtccttgtcggaggtcacgaccagggtgtggccgttggattcgagatattcgcgcaggccgagctcgccggagacggagccgagcaactgcccgggcgtgaagtcgatggccttcggcgtcggcaagatctggccgcccggatagtggtcgatcttcggaagatcgtcgcgggcataggtcttcgggtagccgtcgaccggatcatcgtaaagaacgcacaggacctttgccatcatatgtatatctccttcttaaagttaaacaaaattatttctagaggggaattgttatccgctcacaattcccctatagtgagtcgtattaatttcgcgggatcgagatctcgatcctctacgccggacgcatcgtggccggcatcaccggcgccacaggtgcggttgctggcgcctatatcgccgacatcaccgatggggaagatcgggctcgccacttcgggctcatgagcgcttgtttcggcgtgggtatggtggcaggccccgtggccgggggactgttgggcgccatctccttgcatgcaccattccttgcggcggcggtgctcaacggcctcaacctactactgggctgcttcctaatgcaggagtcgcataagggagagcgtcgagatcccggacaccatcgaatggcgcaaaacctttcgcggtatggcatgatagcgcccggaagagagtcaattcagggtggtgaatgtgaaaccagtaacgttatacgatgtcgcagagtatgccggtgtctcttatcagaccgtttcccgcgtggtgaaccaggccagccacgtttctgcgaaaacgcgggaaaaagtggaagcggcgatggcggagctgaattacattcccaaccgcgtggcacaacaactggcgggcaaacagtcgttgctgattggcgttgccacctccagtctggccctgcacgcgccgtcgcaaattgtcgcggcgattaaatctcgcgccgatcaactgggtgccagcgtggtggtgtcgatggtagaacgaagcggcgtcgaagcctgtaaagcggcggtgcacaatcttctcgcgcaacgcgtcagtgggctgatcattaactatccgctggatgaccaggatgccattgctgtggaagctgcctgcactaatgttccggcgttatttcttgatgtctctgaccagacacccatcaacagtattattttctcccatgaagacggtacgcgactgggcgtggagcatctggtcgcattgggtcaccagcaaatcgcgctgttagcgggcccattaagttctgtctcggcgcgtctgcgtctggctggctggcataaatatctcactcgcaatcaaattcagccgatagcggaacgggaaggcgactggagtgccatgtccggttttcaacaaaccatgcaaatgctgaatgagggcatcgttcccactgcgatgctggttgccaacgatcagatggcgctgggcgcaatgcgcgccattaccgagtccgggctgcgcgttggtgcggatatctcggtagtgggatacgacgataccgaagacagctcatgttatatcccgccgttaaccaccatcaaacaggattttcgcctgctggggcaaaccagcgtggaccgcttgctgcaactctctcagggccaggcggtgaagggcaatcagctgttgcccgtctcactggtgaaaagaaaaaccaccctggcgcccaatacgcaaaccgcctctccccgcgcgttggccgattcattaatgcagctggcacgacaggtttcccgactggaaagcgggcagtgagcgcaacgcaattaatgtaagttagctcactcattaggcaccgggatctcgaccgatgcccttgagagccttcaacccagtcagctccttccggtgggcgcggggcatgactatcgtcgccgcacttatgactgtcttctttatcatgcaactcgtaggacaggtgccggcagcgctctgggtcattttcggcgaggaccgctttcgctggagcgcgacgatgatcggcctgtcgcttgcggtattcggaatcttgcacgccctcgctcaagccttcgtcactggtcccgccaccaaacgtttcggcgagaagcaggccattatcgccggcatggcggccccacgggtgcgcatgatcgtgctcctgtcgttgaggacccggctaggctggcggggttgccttactggttagcagaatgaatcaccgatacgcgagcgaacgtgaagcgactgctgctgcaaaacgtctgcgacctgagcaacaacatgaatggtcttcggtttccgtgtttcgtaaagtctggaaacgcggaagtcagcgccctgcaccattatgttccggatctgcatcgcaggatgctgctggctaccctgtggaacacctacatctgtattaacgaagcgctggcattgaccctgagtgatttttctctggtcccgccgcatccataccgccagttgtttaccctcacaacgttccagtaaccgggcatgttcatcatcagtaacccgtatcgtgagcatcctctctcgtttcatcggtatcattacccccatgaacagaaatcccccttacacggaggcatcagtgaccaaacaggaaaaaaccgcccttaacatggcccgctttatcagaagccagacattaacgcttctggagaaactcaacgagctggacgcggatgaacaggcagacatctgtgaatcgcttcacgaccacgctgatgagctttaccgcagctgcctcgcgcgtttcggtgatgacggtgaaaacctctgacacatgcagctcccggagacggtcacagcttgtctgtaagcggatgccgggagcagacaagcccgtcagggcgcgtcagcgggtgttggcgggtgtcggggcgcagccatgacccagtcacgtagcgatagcggagtgtatactggcttaactatgcggcatcagagcagattgtactgagagtgcaccatatatgcggtgtgaaataccgcacagatgcgtaaggagaaaataccgcatcaggcgctcttccgcttcctcgctcactgactcgctgcgctcggtcgttcggctgcggcgagcggtatcagctcactcaaaggcggtaatacggttatccacagaatcaggggataacgcaggaaagaacatgtgagcaaaaggccagcaaaaggccaggaaccgtaaaaaggccgcgttgctggcgtttttccataggctccgcccccctgacgagcatcacaaaaatcgacgctcaagtcagaggtggcgaaacccgacaggactataaagataccaggcgtttccccctggaagctccctcgtgcgctctcctgttccgaccctgccgcttaccggatacctgtccgcctttctcccttcgggaagcgtggcgctttctcatagctcacgctgtaggtatctcagttcggtgtaggtcgttcgctccaagctgggctgtgtgcacgaaccccccgttcagcccgaccgctgcgccttatccggtaactatcgtcttgagtccaacccggtaagacacgacttatcgccactggcagcagccactggtaacaggattagcagagcgaggtatgtaggcggtgctacagagttcttgaagtggtggcctaactacggctacactagaaggacagtatttggtatctgcgctctgctgaagccagttaccttcggaaaaagagttggtagctcttgatccggcaaacaaaccaccgctggtagcggtggtttttttgtttgcaagcagcagattacgcgcagaaaaaaaggatctcaagaagatcctttgatcttttctacggggtctgacgctcagtggaacgaaaactcacgttaagggattttggtcatgagattatcaaaaaggatcttcacctagatccttttaaattaaaaatgaagttttaaatcaatctaaagtatatatgagtaaacttggtctgacagttaccaatgcttaatcagtgaggcacctatctcagcgatctgtctatttcgttcatccatagttgcctgactccccgtcgtgtagataactacgatacgggagggcttaccatctggccccagtgctgcaatgataccgcgagacccacgctcaccggctccagatttatcagcaataaaccagccagccggaagggccgagcgcagaagtggtcctgcaactttatccgcctccatccagtctattaattgttgccgggaagctagagtaagtagttcgccagttaatagtttgcgcaacgttgttgccattgctgcaggcatcgtggtgtcacgctcgtcgtttggtatggcttcattcagctccggttcccaacgatcaaggcgagttacatgatcccccatgttgtgcaaaaaagcggttagctccttcggtcctccgatcgttgtcagaagtaagttggccgcagtgttatcactcatggttatggcagcactgcataattctcttactgtcatgccatccgtaagatgcttttctgtgactggtgagtactcaaccaagtcattctgagaatagtgtatgcggcgaccgagttgctcttgcccggcgtcaatacgggataataccgcgccacatagcagaactttaaaagtgctcatcattggaaaacgttcttcggggcgaaaactctcaaggatcttaccgctgttgagatccagttcgatgtaacccactcgtgcacccaactgatcttcagcatcttttactttcaccagcgtttctgggtgagcaaaaacaggaaggcaaaatgccgcaaaaaagggaataagggcgacacggaaatgttgaatactcatactcttcctttttcaatattattgaagcatttatcagggttattgtctcatgagcggatacatatttgaatgtatttagaaaaataaacaaataggggttccgcgcacatttccccgaaaagtgccacctgaaattgtaaacgttaatattttgttaaaattcgcgttaaatttttgttaaatcagctcattttttaaccaataggccgaaatcggcaaaatcccttataaatcaaaagaatagaccgagatagggttgagtgttgttccagtttggaacaagagtccactattaaagaacgtggactccaacgtcaaagggcgaaaaaccgtctatcagggcgatggcccactacgtgaaccatcaccctaatcaagttttttggggtcgaggtgccgtaaagcactaaatcggaaccctaaagggagcccccgatttagagcttgacggggaaagccggcgaacgtggcgagaaaggaagggaagaaagcgaaaggagcgggcgctagggcgctggcaagtgtagcggtcacgctgcgcgtaaccaccacacccgccgcgcttaatgcgccgctacagggcgcgtcccattcgcca

SEQ ID NO: 52 - DNA, 7404 bp, artificial
  Vektor pFr7(DV)
atccggatatagttcctcctttcagcaaaaaacccctcaagacccgtttagaggccccaaggggttatgctagttattgctcagcggtggcagcagccaactcagcttcctttcgggctttgttagcagccggatctcagtggtggtggtggtggtgctcgagtgcggccgcaagcttctagtcgcggtagaacgaccccatgtagcggatgtactcgtcctcggtgtggtttgccttccagtcgtggacggagtccttgttgcgctggccggcgatgacggagagctccttacccagcttctcaaaggcctcgtcaacgcactcctcgggggtgagggcgatcttcatgacggcctcgccctgcgggccgccggggaggttggacagcaggctgggggttagggtggtgccgagggtgatgacctcgacgtcgacgccggtgccctcgcactcgcaggccacggcctcggtcatcttgaggatgaaggccttgcccgcgccgtactggccgttccaggggctggagctgatgccggtcatcgacgagacgttgatcacggcgccgcggtcctgggcggcaaagatccgcatgtagtggtggaagcacttgaggaaggtcacgacgttgacgttgatcatggcctcgtgcttctcccagggggtgtcctggatcttaccgaagctgtgcaggcaggccacgtagctcatgaagcccatgtccaggccctcggtcgcggcgaagacggtctcggcagcgccgggctggctaaagtcggcgcgcacgaccttggtctccacgccgtaggtctcgcggatctcgcctgcgagcacgttcagcttctcctcgcgaacgtcgaccatgacgacgttcatgccgccggcggcgatcttctcgcagaacgccttgccgacgccctcggtcgcgcccaggatcaggccccactcaccgtacttctccctcaggttcatgtatatctcctttcacgaattctcagccgccttcttgaacttggcggcctcttccgaaccgccggtggcattgcccttcgagtaggaatgcgcgccggtgccggcaagagcgccgccctgcacgatgaggtattcgtcgcggatcggacggccctcgaagaagcactccaggatctcgcgggtgcccgccgcataacgcgcctgcgcggtcagcgtggtgccggagatgtgcggggtcatgccgttatagggcatcgtccgccaggggtggtccttcggcgccggctgcgggaaccacacgtcgccggcatagccggccagccggccggattcgagcgcacgtgccacggcatcgcggtcgcacagcttgccgcgggcggtgttgacgatgtaggcgccacgcttgaacagcttcagcgtctcgtcattgatcatgtgctcggtttcggggtgcagcgggcagttcagcgtcaccacgtcgcaaaccggatacatgtcctcgcgggtcgcgtgccaggtgaggttgagctccttctcgaccgattccggcaggcggtgacggccggtgtagtgcaggtgcacgtcgaacggcgccagacggcgcagcaccgcgagaccgatgcggccggcggccacggtgccgacatgcatcgcctcgaggtcgtaggcgtgggagacgcagtcggcgatgttccagccgcccttccgcgcccattcgtgcgagggcagatagttgcgcaccagcgacaggatcatcatcaccacatgctcggcgacgctgatcgagttgcagtaggtgacttccgccacggtgacgttgcggtcgatagccgactgaagatcgacgtggtcggaaccgatgccggcggtgagcgcgagcttcaggttcttggccttggcgatgcgctcgggcgtcagataggccggccagaagggctgggagatgacgacatccgcatcgaccagctcgcgctcgaacaccgagtcggggccgtccttgtcggaggtcacgaccagggtgtggccgttggattcgagatattcgcgcaggccgagctcgccggagacggagccgagcaactgcccgggcgtgaagtcgatggccttcggcgtcggcaagatctggccgcccggatagtggtcgatcttcggaagatcgtcgcgggcataggtcttcgggtagccgtcgaccggatcatcgtaaagaacgcacaggacctttgccatcatatgtatatctccttcttaaagttaaacaaaattatttctagaggggaattgttatccgctcacaattcccctatagtgagtcgtattaatttcgcgggatcgagatctcgatcctctacgccggacgcatcgtggccggcatcaccggcgccacaggtgcggttgctggcgcctatatcgccgacatcaccgatggggaagatcgggctcgccacttcgggctcatgagcgcttgtttcggcgtgggtatggtggcaggccccgtggccgggggactgttgggcgccatctccttgcatgcaccattccttgcggcggcggtgctcaacggcctcaacctactactgggctgcttcctaatgcaggagtcgcataagggagagcgtcgagatcccggacaccatcgaatggcgcaaaacctttcgcggtatggcatgatagcgcccggaagagagtcaattcagggtggtgaatgtgaaaccagtaacgttatacgatgtcgcagagtatgccggtgtctcttatcagaccgtttcccgcgtggtgaaccaggccagccacgtttctgcgaaaacgcgggaaaaagtggaagcggcgatggcggagctgaattacattcccaaccgcgtggcacaacaactggcgggcaaacagtcgttgctgattggcgttgccacctccagtctggccctgcacgcgccgtcgcaaattgtcgcggcgattaaatctcgcgccgatcaactgggtgccagcgtggtggtgtcgatggtagaacgaagcggcgtcgaagcctgtaaagcggcggtgcacaatcttctcgcgcaacgcgtcagtgggctgatcattaactatccgctggatgaccaggatgccattgctgtggaagctgcctgcactaatgttccggcgttatttcttgatgtctctgaccagacacccatcaacagtattattttctcccatgaagacggtacgcgactgggcgtggagcatctggtcgcattgggtcaccagcaaatcgcgctgttagcgggcccattaagttctgtctcggcgcgtctgcgtctggctggctggcataaatatctcactcgcaatcaaattcagccgatagcggaacgggaaggcgactggagtgccatgtccggttttcaacaaaccatgcaaatgctgaatgagggcatcgttcccactgcgatgctggttgccaacgatcagatggcgctgggcgcaatgcgcgccattaccgagtccgggctgcgcgttggtgcggatatctcggtagtgggatacgacgataccgaagacagctcatgttatatcccgccgttaaccaccatcaaacaggattttcgcctgctggggcaaaccagcgtggaccgcttgctgcaactctctcagggccaggcggtgaagggcaatcagctgttgcccgtctcactggtgaaaagaaaaaccaccctggcgcccaatacgcaaaccgcctctccccgcgcgttggccgattcattaatgcagctggcacgacaggtttcccgactggaaagcgggcagtgagcgcaacgcaattaatgtaagttagctcactcattaggcaccgggatctcgaccgatgcccttgagagccttcaacccagtcagctccttccggtgggcgcggggcatgactatcgtcgccgcacttatgactgtcttctttatcatgcaactcgtaggacaggtgccggcagcgctctgggtcattttcggcgaggaccgctttcgctggagcgcgacgatgatcggcctgtcgcttgcggtattcggaatcttgcacgccctcgctcaagccttcgtcactggtcccgccaccaaacgtttcggcgagaagcaggccattatcgccggcatggcggccccacgggtgcgcatgatcgtgctcctgtcgttgaggacccggctaggctggcggggttgccttactggttagcagaatgaatcaccgatacgcgagcgaacgtgaagcgactgctgctgcaaaacgtctgcgacctgagcaacaacatgaatggtcttcggtttccgtgtttcgtaaagtctggaaacgcggaagtcagcgccctgcaccattatgttccggatctgcatcgcaggatgctgctggctaccctgtggaacacctacatctgtattaacgaagcgctggcattgaccctgagtgatttttctctggtcccgccgcatccataccgccagttgtttaccctcacaacgttccagtaaccgggcatgttcatcatcagtaacccgtatcgtgagcatcctctctcgtttcatcggtatcattacccccatgaacagaaatcccccttacacggaggcatcagtgaccaaacaggaaaaaaccgcccttaacatggcccgctttatcagaagccagacattaacgcttctggagaaactcaacgagctggacgcggatgaacaggcagacatctgtgaatcgcttcacgaccacgctgatgagctttaccgcagctgcctcgcgcgtttcggtgatgacggtgaaaacctctgacacatgcagctcccggagacggtcacagcttgtctgtaagcggatgccgggagcagacaagcccgtcagggcgcgtcagcgggtgttggcgggtgtcggggcgcagccatgacccagtcacgtagcgatagcggagtgtatactggcttaactatgcggcatcagagcagattgtactgagagtgcaccatatatgcggtgtgaaataccgcacagatgcgtaaggagaaaataccgcatcaggcgctcttccgcttcctcgctcactgactcgctgcgctcggtcgttcggctgcggcgagcggtatcagctcactcaaaggcggtaatacggttatccacagaatcaggggataacgcaggaaagaacatgtgagcaaaaggccagcaaaaggccaggaaccgtaaaaaggccgcgttgctggcgtttttccataggctccgcccccctgacgagcatcacaaaaatcgacgctcaagtcagaggtggcgaaacccgacaggactataaagataccaggcgtttccccctggaagctccctcgtgcgctctcctgttccgaccctgccgcttaccggatacctgtccgcctttctcccttcgggaagcgtggcgctttctcatagctcacgctgtaggtatctcagttcggtgtaggtcgttcgctccaagctgggctgtgtgcacgaaccccccgttcagcccgaccgctgcgccttatccggtaactatcgtcttgagtccaacccggtaagacacgacttatcgccactggcagcagccactggtaacaggattagcagagcgaggtatgtaggcggtgctacagagttcttgaagtggtggcctaactacggctacactagaaggacagtatttggtatctgcgctctgctgaagccagttaccttcggaaaaagagttggtagctcttgatccggcaaacaaaccaccgctggtagcggtggtttttttgtttgcaagcagcagattacgcgcagaaaaaaaggatctcaagaagatcctttgatcttttctacggggtctgacgctcagtggaacgaaaactcacgttaagggattttggtcatgagattatcaaaaaggatcttcacctagatccttttaaattaaaaatgaagttttaaatcaatctaaagtatatatgagtaaacttggtctgacagttaccaatgcttaatcagtgaggcacctatctcagcgatctgtctatttcgttcatccatagttgcctgactccccgtcgtgtagataactacgatacgggagggcttaccatctggccccagtgctgcaatgataccgcgagacccacgctcaccggctccagatttatcagcaataaaccagccagccggaagggccgagcgcagaagtggtcctgcaactttatccgcctccatccagtctattaattgttgccgggaagctagagtaagtagttcgccagttaatagtttgcgcaacgttgttgccattgctgcaggcatcgtggtgtcacgctcgtcgtttggtatggcttcattcagctccggttcccaacgatcaaggcgagttacatgatcccccatgttgtgcaaaaaagcggttagctccttcggtcctccgatcgttgtcagaagtaagttggccgcagtgttatcactcatggttatggcagcactgcataattctcttactgtcatgccatccgtaagatgcttttctgtgactggtgagtactcaaccaagtcattctgagaatagtgtatgcggcgaccgagttgctcttgcccggcgtcaatacgggataataccgcgccacatagcagaactttaaaagtgctcatcattggaaaacgttcttcggggcgaaaactctcaaggatcttaccgctgttgagatccagttcgatgtaacccactcgtgcacccaactgatcttcagcatcttttactttcaccagcgtttctgggtgagcaaaaacaggaaggcaaaatgccgcaaaaaagggaataagggcgacacggaaatgttgaatactcatactcttcctttttcaatattattgaagcatttatcagggttattgtctcatgagcggatacatatttgaatgtatttagaaaaataaacaaataggggttccgcgcacatttccccgaaaagtgccacctgaaattgtaaacgttaatattttgttaaaattcgcgttaaatttttgttaaatcagctcattttttaaccaataggccgaaatcggcaaaatcccttataaatcaaaagaatagaccgagatagggttgagtgttgttccagtttggaacaagagtccactattaaagaacgtggactccaacgtcaaagggcgaaaaaccgtctatcagggcgatggcccactacgtgaaccatcaccctaatcaagttttttggggtcgaggtgccgtaaagcactaaatcggaaccctaaagggagcccccgatttagagcttgacggggaaagccggcgaacgtggcgagaaaggaagggaagaaagcgaaaggagcgggcgctagggcgctggcaagtgtagcggtcacgctgcgcgtaaccaccacacccgccgcgcttaatgcgccgctacagggcgcgtcccattcgcca

SEQ ID NO: 53 - DNA, 27 bp, artificial
  PCR Primer "G39D for"
gtcgtcatggtcgaccgtcgcgaggag

SEQ ID NO: 54 - DNA, 27 bp, artificial
  PCR Primer "G39D_rev"
ctcctcgcgacggtcgaccatgacgac

SEQ ID NO: 55 - DNA, 24 bp, artificial
  PCR Primer "G39D/R40I_for"
gtcatggtcgacattcgcgaggag

SEQ ID NO: 56 - DNA, 24 bp, artificial
  PCR Primer "G39D/R40I_rev"
ctcctcgcgaatgtcgaccatgac

SEQ ID NO: 57 - DNA, 27 bp, artificial
  PCR Primer "R40D_for"
gtcatggtcggcgatcgcgaggagaag

SEQ ID NO: 58 - DNA, 27 bp, artificial
  PCR Primer "R40D_rev"
cttctcctcgcgatcgccgaccatgac

SEQ ID NO: 59 - DNA, 30 bp, artificial
  PCR Primer "R40D/R41I_for"
gtcatggtcggcgatatcgaggagaagctg

SEQ ID NO: 60 - DNA, 30 bp, artificial
  PCR Primer "R40D/R41I_rev"
cagcttctcctcgatatcgccgaccatgac

SEQ ID NO: 61 - DNA, 27 bp, artificial
  PCR Primer "DIN_for"
atggtcgacattaacgaggagaagctg

SEQ ID NO: 62 - DNA, 27 bp, artificial
  PCR Primer "DIN_rev"
cagcttctcctcgttaatgtcgaccat

SEQ ID NO: 63 - DNA, 8321 bp, artificial
  Plasmid pFr3T7(D)
atccggatatagttcctcctttcagcaaaaaacccctcaagacccgtttagaggccccaaggggttatgctagttattgctcagcggtggcagcagccaactcagcttcctttcgggctttgttagcagccggatctcagtggtggtggtggtggtgctcgagtgcggccgcctagtcgcggtagaacgaccccatgtagcggatgtactcgtcctcggtgtggtttgccttccagtcgtggacggagtccttgttgcgctggccggcgatgacggagagctccttacccagcttctcaaaggcctcgtcaacgcactcctcgggggtgagggcgatcttcatgacggcctcgccctgcgggccgccggggaggttggacagcaggctgggggttagggtggtgccgagggtgatgacctcgacgtcgacgccggtgccctcgcactcgcaggccacggcctcggtcatcttgaggatgaaggccttgcccgcgccgtactggccgttccaggggctggagctgatgccggtcatcgacgagacgttgatcacggcgccgcggtcctgggcggcaaagatccgcatgtagtggtggaagcacttgaggaaggtcacgacgttgacgttgatcatggcctcgtgcttctcccagggggtgtcctggatcttaccgaagctgtgcaggcaggccacgtagctcatgaagcccatgtccaggccctcggtcgcggcgaagacggtctcggcagcgccgggctggctaaagtcggcgcgcacgaccttggtctccacgccgtaggtctcgcggatctcgcctgcgagcacgttcagcttctcctcgcgacggtcgaccatgacgacgttcatgccgccggcggcgatcttctcgcagaacgccttgccgacgccctcggtcgcgcccaggatcaggccccactcaccgtacttctccctcaggttcatatgtatatctccttcttatacttaactaatatactaagatggggaattgttatccgctcacaattcccctatagtgagtcgtattaatttcgattatgcggccgtgtacaatacgattactttctgttcgacttaagcattataagctttcagaactgtgtcgggcgcatcaccgcatcaatgccgccatcaatgacgatctgcgcgccatgcacatagcttgcggccgggctcatcaaaaaggcgatgaccgacgccatctcggacggctcggcacggcggcccatgggaggaacgaacttggcaatggattcgccatagcgcgggtcctgcaggcccgcctgcagcaagggagtctcggttgcaccgggggcgatggtgttcaggcgcacgccagcctcgccccaggcggcggcgcgtttgcgcacagccaccgtcaaagcattcttgctgcccgcataggccagatttccgccctgctctcccgcatgttcgacaatggcgcgggccttggcttcctcgccggcttccagtgccagcgccagtgggttcttgtcaaaagccagatgcgcggaagccacggacgagatgacgacggctgcgggctgatggccttttttcagcgctggcaaaaaggcatccatcagctcggtcgcgccaaaataattgaccgaaaccacattgccaagcaccttggtctgcggtcccaggccggcgcacagcaccaggccgtccatgcccttgctgcacttcgccagtacatcggcaatcgcctgctttcgaccttcggccgtcgagagatcggcaatcacttccgcatcgcgtatatcgatgcctacgatctggtgaccggccgcctccaggaccttgcgcgtagccgcaccaatgccggtggcgcagccgcttatcacgatgatggacatgtatatctcctttcacgaattctcagccgccttcttgaacttggcggcctcttccgaaccgccggtggcattgcccttcgagtaggaatgcgcgccggtgccggcaagagcgccgccctgcacgatgaggtattcgtcgcggatcggacggccctcgaagaagcactccaggatctcgcgggtgcccgccgcataacgcgcctgcgcggtcagcgtggtgccggagatgtgcggggtcatgccgttatagggcatcgtccgccaggggtggtccttcggcgccggctgcgggaaccacacgtcgccggcatagccggccagccggccggattcgagcgcacgtgccacggcatcgcggtcgcacagcttgccgcgggcggtgttgacgatgtaggcgccacgcttgaacagcttcagcgtctcgtcattgatcatgtgctcggtttcggggtgcagcgggcagttcagcgtcaccacgtcgcaaaccggatacatgtcctcgcgggtcgcgtgccaggtgaggttgagctccttctcgaccgattccggcaggcggtgacggtcggtgtagtgcaggtgcacgtcgaacggcgccagacggcgcagcaccgcgagaccgatgcggccggcggccacggtgccgacatgcatcgcctcgaggtcgtaggcgtgggagacgcagtcggcgatgttccagccgcccttccgcgcccattcgtgcgagggcagatagttgcgcaccagcgacaggatcatcatcaccacatgctcggcgacgctgatcgagttgcagtaggtgacttccgccacggtgacgttgcggtcgatagccgactgaagatcgacgtggtcggaaccgatgccggcggtgagcgcgagcttcaggttcttggccttggcgatgcgctcgggcgtcagataggccggccagaagggctgggagatgacgacatccgcatcgaccagctcgcgctcgaacaccgagtcggggccgtccttgtcggaggtcacgaccagggtgtggccgttggattcgagatattcgcgcaggccgagctcgccggagacggagccgagcaactgcccgggcgtgaagtcgatggccttcggcgtcggcaagatctggccgcccggatagtggtcgatcttcggaagatcgtcgcgggcataggtcttcgggtagccgtcgaccggatcatcgtaaagaacgcacaggacctttgccatcatatgtatatctccttcttaaagttaaacaaaattatttctagaggggaattgttatccgctcacaattcccctatagtgagtcgtattaatttcgcgggatcgagatctcgatcctctacgccggacgcatcgtggccggcatcaccggcgccacaggtgcggttgctggcgcctatatcgccgacatcaccgatggggaagatcgggctcgccacttcgggctcatgagcgcttgtttcggcgtgggtatggtggcaggccccgtggccgggggactgttgggcgccatctccttgcatgcaccattccttgcggcggcggtgctcaacggcctcaacctactactgggctgcttcctaatgcaggagtcgcataagggagagcgtcgagatcccggacaccatcgaatggcgcaaaacctttcgcggtatggcatgatagcgcccggaagagagtcaattcagggtggtgaatgtgaaaccagtaacgttatacgatgtcgcagagtatgccggtgtctcttatcagaccgtttcccgcgtggtgaaccaggccagccacgtttctgcgaaaacgcgggaaaaagtggaagcggcgatggcggagctgaattacattcccaaccgcgtggcacaacaactggcgggcaaacagtcgttgctgattggcgttgccacctccagtctggccctgcacgcgccgtcgcaaattgtcgcggcgattaaatctcgcgccgatcaactgggtgccagcgtggtggtgtcgatggtagaacgaagcggcgtcgaagcctgtaaagcggcggtgcacaatcttctcgcgcaacgcgtcagtgggctgatcattaactatccgctggatgaccaggatgccattgctgtggaagctgcctgcactaatgttccggcgttatttcttgatgtctctgaccagacacccatcaacagtattattttctcccatgaagacggtacgcgactgggcgtggagcatctggtcgcattgggtcaccagcaaatcgcgctgttagcgggcccattaagttctgtctcggcgcgtctgcgtctggctggctggcataaatatctcactcgcaatcaaattcagccgatagcggaacgggaaggcgactggagtgccatgtccggttttcaacaaaccatgcaaatgctgaatgagggcatcgttcccactgcgatgctggttgccaacgatcagatggcgctgggcgcaatgcgcgccattaccgagtccgggctgcgcgttggtgcggatatctcggtagtgggatacgacgataccgaagacagctcatgttatatcccgccgttaaccaccatcaaacaggattttcgcctgctggggcaaaccagcgtggaccgcttgctgcaactctctcagggccaggcggtgaagggcaatcagctgttgcccgtctcactggtgaaaagaaaaaccaccctggcgcccaatacgcaaaccgcctctccccgcgcgttggccgattcattaatgcagctggcacgacaggtttcccgactggaaagcgggcagtgagcgcaacgcaattaatgtaagttagctcactcattaggcaccgggatctcgaccgatgcccttgagagccttcaacccagtcagctccttccggtgggcgcggggcatgactatcgtcgccgcacttatgactgtcttctttatcatgcaactcgtaggacaggtgccggcagcgctctgggtcattttcggcgaggaccgctttcgctggagcgcgacgatgatcggcctgtcgcttgcggtattcggaatcttgcacgccctcgctcaagccttcgtcactggtcccgccaccaaacgtttcggcgagaagcaggccattatcgccggcatggcggccccacgggtgcgcatgatcgtgctcctgtcgttgaggacccggctaggctggcggggttgccttactggttagcagaatgaatcaccgatacgcgagcgaacgtgaagcgactgctgctgcaaaacgtctgcgacctgagcaacaacatgaatggtcttcggtttccgtgtttcgtaaagtctggaaacgcggaagtcagcgccctgcaccattatgttccggatctgcatcgcaggatgctgctggctaccctgtggaacacctacatctgtattaacgaagcgctggcattgaccctgagtgatttttctctggtcccgccgcatccataccgccagttgtttaccctcacaacgttccagtaaccgggcatgttcatcatcagtaacccgtatcgtgagcatcctctctcgtttcatcggtatcattacccccatgaacagaaatcccccttacacggaggcatcagtgaccaaacaggaaaaaaccgcccttaacatggcccgctttatcagaagccagacattaacgcttctggagaaactcaacgagctggacgcggatgaacaggcagacatctgtgaatcgcttcacgaccacgctgatgagctttaccgcagctgcctcgcgcgtttcggtgatgacggtgaaaacctctgacacatgcagctcccggagacggtcacagcttgtctgtaagcggatgccgggagcagacaagcccgtcagggcgcgtcagcgggtgttggcgggtgtcggggcgcagccatgacccagtcacgtagcgatagcggagtgtatactggcttaactatgcggcatcagagcagattgtactgagagtgcaccatatatgcggtgtgaaataccgcacagatgcgtaaggagaaaataccgcatcaggcgctcttccgcttcctcgctcactgactcgctgcgctcggtcgttcggctgcggcgagcggtatcagctcactcaaaggcggtaatacggttatccacagaatcaggggataacgcaggaaagaacatgtgagcaaaaggccagcaaaaggccaggaaccgtaaaaaggccgcgttgctggcgtttttccataggctccgcccccctgacgagcatcacaaaaatcgacgctcaagtcagaggtggcgaaacccgacaggactataaagataccaggcgtttccccctggaagctccctcgtgcgctctcctgttccgaccctgccgcttaccggatacctgtccgcctttctcccttcgggaagcgtggcgctttctcatagctcacgctgtaggtatctcagttcggtgtaggtcgttcgctccaagctgggctgtgtgcacgaaccccccgttcagcccgaccgctgcgccttatccggtaactatcgtcttgagtccaacccggtaagacacgacttatcgccactggcagcagccactggtaacaggattagcagagcgaggtatgtaggcggtgctacagagttcttgaagtggtggcctaactacggctacactagaaggacagtatttggtatctgcgctctgctgaagccagttaccttcggaaaaagagttggtagctcttgatccggcaaacaaaccaccgctggtagcggtggtttttttgtttgcaagcagcagattacgcgcagaaaaaaaggatctcaagaagatcctttgatcttttctacggggtctgacgctcagtggaacgaaaactcacgttaagggattttggtcatgagattatcaaaaaggatcttcacctagatccttttaaattaaaaatgaagttttaaatcaatctaaagtatatatgagtaaacttggtctgacagttaccaatgcttaatcagtgaggcacctatctcagcgatctgtctatttcgttcatccatagttgcctgactccccgtcgtgtagataactacgatacgggagggcttaccatctggccccagtgctgcaatgataccgcgagacccacgctcaccggctccagatttatcagcaataaaccagccagccggaagggccgagcgcagaagtggtcctgcaactttatccgcctccatccagtctattaattgttgccgggaagctagagtaagtagttcgccagttaatagtttgcgcaacgttgttgccattgctgcaggcatcgtggtgtcacgctcgtcgtttggtatggcttcattcagctccggttcccaacgatcaaggcgagttacatgatcccccatgttgtgcaaaaaagcggttagctccttcggtcctccgatcgttgtcagaagtaagttggccgcagtgttatcactcatggttatggcagcactgcataattctcttactgtcatgccatccgtaagatgcttttctgtgactggtgagtactcaaccaagtcattctgagaatagtgtatgcggcgaccgagttgctcttgcccggcgtcaatacgggataataccgcgccacatagcagaactttaaaagtgctcatcattggaaaacgttcttcggggcgaaaactctcaaggatcttaccgctgttgagatccagttcgatgtaacccactcgtgcacccaactgatcttcagcatcttttactttcaccagcgtttctgggtgagcaaaaacaggaaggcaaaatgccgcaaaaaagggaataagggcgacacggaaatgttgaatactcatactcttcctttttcaatattattgaagcatttatcagggttattgtctcatgagcggatacatatttgaatgtatttagaaaaataaacaaataggggttccgcgcacatttccccgaaaagtgccacctgaaattgtaaacgttaatattttgttaaaattcgcgttaaatttttgttaaatcagctcattttttaaccaataggccgaaatcggcaaaatcccttataaatcaaaagaatagaccgagatagggttgagtgttgttccagtttggaacaagagtccactattaaagaacgtggactccaacgtcaaagggcgaaaaaccgtctatcagggcgatggcccactacgtgaaccatcaccctaatcaagttttttggggtcgaggtgccgtaaagcactaaatcggaaccctaaagggagcccccgatttagagcttgacggggaaagccggcgaacgtggcgagaaaggaagggaagaaagcgaaaggagcgggcgctagggcgctggcaagtgtagcggtcacgctgcgcgtaaccaccacacccgccgcgcttaatgcgccgctacagggcgcgtcccattcgcca

SEQ ID NO: 64 - DNA, 8190 bp, artificial
  pF(G)r7(A)r3
atccggatatagttcctcctttcagcaaaaaacccctcaagacccgtttagaggccccaaggggttatgctagttattgctcagcggtggcagcagccaactcagcttcctttcgggctttgttagcagccggatctcagtggtggtggtggtggtgctcgagtgcggccgctcagaactgtgtcgggcgcatcaccgcatcaatgccgccatcaatgacgatctgcgcgccatgcacatagcttgcggccgggctcatcaaaaaggcgatgaccgacgccatctcggacggctcggcacggcggcccatgggaggaacgaacttggcaatggattcgccatagcgcgggtcctgcaggcccgcctgcagcaagggagtctcggttgcaccgggggcgatggtgttcaggcgcacgccagcctcgccccaggcggcggcgcgtttgcgcacagccaccgtcaaagcattcttgctgcccgcataggccagatttccgccctgctctcccgcatgttcgacaatggcgcgggccttggcttcctcgccggcttccagtgccagcgccagtgggttcttgtcaaaagccagatgcgcggaagccacggacgagatgacgacggctgcgggctgatggccttttttcagcgctggcaaaaaggcatccatcagctcggtcgcgccaaaataattgaccgaaaccacattgccaagcaccttggtctgcggtcccaggccggcgcacagcaccaggccgtccatgcccttgctgcacttcgccagtacatcggcaatcgcctgctttcgaccttcggccgtcgagagatcggcaatcacttccgcatcgcgtatatcgatgcctacgatctggtgaccggccgcctccaggaccttgcgcgtagcggcaccaatgccggtggcgcagccgcttatcacgatgatggacatgtatatctccttaagcttctagtcgcggtagaacgaccccatgtagcggatgtactcgtcctcggtgtggtttgccttccagtcgtggacggagtccttgttgcgctggccggcgatgacggagagctccttacccagcttctcaaaggcctcgtcaacgcactcctcgggggtgagggcgatcttcatgacggcctcgccctgcgggccgccggggaggttggacagcaggctgggggttagggtggtgccgagggtgatgacctcgacgtcgacgccggtgccctcgcactcgcaggccacggcctcggtcatcttgaggatgaaggccttgcccgcgccgtactggccgttccaggggctggagctgatgccggtcatcgacgagacgttgatcacggcgccgcggtcctgggcggcaaagatccgcatgtagtggtggaagcacttgaggaaggtcacgacgttgacgttgatcatggcctcgtgcttctcccagggggtgtcctggatcttaccgaagctgtgcaggcaggccacgtagctcatgaagcccatgtccaggccctcggtcgcggcgaagacggtctcggcagcgccgggctggctaaagtcggcgcgcacgaccttggtctccacgccgtaggtctcgcggatctcgcctgcgagcacgttcagcttctcctcgcgacgggcgaccatgacgacgttcatgccgccggcggcgatcttctcgcagaacgccttgccgacgccctcggtcgcgcccaggatcaggccccactcaccgtacttctccctcaggttcatgtatatctcctttcacgaattctcagccgccttcttgaacttggcggcctcttccgaaccgccggtggcattgcccttcgagtaggaatgcgcgccggtgccggcaagagcgccgccctgcacgatgaggtattcgtcgcggatcggacggccctcgaagaagcactccaggatctcgcgggtgcccgccgcataacgcgcctgcgcggtcagcgtggtgccggagatgtgcggggtcatgccgttatagggcatcgtccgccaggggtggtccttcggcgccggctgcgggaaccacacgtcgccggcatagccggccagccggccggattcgagcgcacgtgccacggcatcgcggtcgcacagcttgccgcgggcggtgttgacgatgtaggcgccacgcttgaacagcttcagcgtctcgtcattgatcatgtgctcggtttcggggtgcagcgggcagttcagcgtcaccacgtcgcaaaccggatacatgtcctcgcgggtcgcgtgccaggtgaggttgagctccttctcgaccgattccggcaggcggtgacggccggtgtagtgcaggtgcacgtcgaacggcgccagacggcgcagcaccgcgagaccgatgcggccggcggccacggtgccgacatgcatcgcctcgaggtcgtaggcgtgggagacgcagtcggcgatgttccagccgcccttccgcgcccattcgtgcgagggcagatagttgcgcaccagcgacaggatcatcatcaccacatgctcggcgacgctgatcgagttgcagtaggtgacttccgccacggtgacgttgcggtcgatagccgactgaagatcgacgtggtcggaaccgatgccggcggtgagcgcgagcttcaggttcttggccttggcgatgcgctcgggcgtcagataggccggccagaagggctgggagatgacgacatccgcatcgaccagctcgcgctcgaacaccgagtcggggccgtccttgtcggaggtcacgaccagggtgtggccgttggattcgagatattcgcgcaggccgagctcgccggagacggagccgagcaactgcccgggcgtgaagtcgatggccttcggcgtcggcaagatctggccgcccggatagtggtcgatcttcggaagatcgtcgcgggcataggtcttcgggtagccgtcgaccggatcatcgtaaagaacgcacaggacctttgccatcatatgtatatctccttcttaaagttaaacaaaattatttctagaggggaattgttatccgctcacaattcccctatagtgagtcgtattaatttcgcgggatcgagatctcgatcctctacgccggacgcatcgtggccggcatcaccggcgccacaggtgcggttgctggcgcctatatcgccgacatcaccgatggggaagatcgggctcgccacttcgggctcatgagcgcttgtttcggcgtgggtatggtggcaggccccgtggccgggggactgttgggcgccatctccttgcatgcaccattccttgcggcggcggtgctcaacggcctcaacctactactgggctgcttcctaatgcaggagtcgcataagggagagcgtcgagatcccggacaccatcgaatggcgcaaaacctttcgcggtatggcatgatagcgcccggaagagagtcaattcagggtggtgaatgtgaaaccagtaacgttatacgatgtcgcagagtatgccggtgtctcttatcagaccgtttcccgcgtggtgaaccaggccagccacgtttctgcgaaaacgcgggaaaaagtggaagcggcgatggcggagctgaattacattcccaaccgcgtggcacaacaactggcgggcaaacagtcgttgctgattggcgttgccacctccagtctggccctgcacgcgccgtcgcaaattgtcgcggcgattaaatctcgcgccgatcaactgggtgccagcgtggtggtgtcgatggtagaacgaagcggcgtcgaagcctgtaaagcggcggtgcacaatcttctcgcgcaacgcgtcagtgggctgatcattaactatccgctggatgaccaggatgccattgctgtggaagctgcctgcactaatgttccggcgttatttcttgatgtctctgaccagacacccatcaacagtattattttctcccatgaagacggtacgcgactgggcgtggagcatctggtcgcattgggtcaccagcaaatcgcgctgttagcgggcccattaagttctgtctcggcgcgtctgcgtctggctggctggcataaatatctcactcgcaatcaaattcagccgatagcggaacgggaaggcgactggagtgccatgtccggttttcaacaaaccatgcaaatgctgaatgagggcatcgttcccactgcgatgctggttgccaacgatcagatggcgctgggcgcaatgcgcgccattaccgagtccgggctgcgcgttggtgcggatatctcggtagtgggatacgacgataccgaagacagctcatgttatatcccgccgttaaccaccatcaaacaggattttcgcctgctggggcaaaccagcgtggaccgcttgctgcaactctctcagggccaggcggtgaagggcaatcagctgttgcccgtctcactggtgaaaagaaaaaccaccctggcgcccaatacgcaaaccgcctctccccgcgcgttggccgattcattaatgcagctggcacgacaggtttcccgactggaaagcgggcagtgagcgcaacgcaattaatgtaagttagctcactcattaggcaccgggatctcgaccgatgcccttgagagccttcaacccagtcagctccttccggtgggcgcggggcatgactatcgtcgccgcacttatgactgtcttctttatcatgcaactcgtaggacaggtgccggcagcgctctgggtcattttcggcgaggaccgctttcgctggagcgcgacgatgatcggcctgtcgcttgcggtattcggaatcttgcacgccctcgctcaagccttcgtcactggtcccgccaccaaacgtttcggcgagaagcaggccattatcgccggcatggcggccccacgggtgcgcatgatcgtgctcctgtcgttgaggacccggctaggctggcggggttgccttactggttagcagaatgaatcaccgatacgcgagcgaacgtgaagcgactgctgctgcaaaacgtctgcgacctgagcaacaacatgaatggtcttcggtttccgtgtttcgtaaagtctggaaacgcggaagtcagcgccctgcaccattatgttccggatctgcatcgcaggatgctgctggctaccctgtggaacacctacatctgtattaacgaagcgctggcattgaccctgagtgatttttctctggtcccgccgcatccataccgccagttgtttaccctcacaacgttccagtaaccgggcatgttcatcatcagtaacccgtatcgtgagcatcctctctcgtttcatcggtatcattacccccatgaacagaaatcccccttacacggaggcatcagtgaccaaacaggaaaaaaccgcccttaacatggcccgctttatcagaagccagacattaacgcttctggagaaactcaacgagctggacgcggatgaacaggcagacatctgtgaatcgcttcacgaccacgctgatgagctttaccgcagctgcctcgcgcgtttcggtgatgacggtgaaaacctctgacacatgcagctcccggagacggtcacagcttgtctgtaagcggatgccgggagcagacaagcccgtcagggcgcgtcagcgggtgttggcgggtgtcggggcgcagccatgacccagtcacgtagcgatagcggagtgtatactggcttaactatgcggcatcagagcagattgtactgagagtgcaccatatatgcggtgtgaaataccgcacagatgcgtaaggagaaaataccgcatcaggcgctcttccgcttcctcgctcactgactcgctgcgctcggtcgttcggctgcggcgagcggtatcagctcactcaaaggcggtaatacggttatccacagaatcaggggataacgcaggaaagaacatgtgagcaaaaggccagcaaaaggccaggaaccgtaaaaaggccgcgttgctggcgtttttccataggctccgcccccctgacgagcatcacaaaaatcgacgctcaagtcagaggtggcgaaacccgacaggactataaagataccaggcgtttccccctggaagctccctcgtgcgctctcctgttccgaccctgccgcttaccggatacctgtccgcctttctcccttcgggaagcgtggcgctttctcatagctcacgctgtaggtatctcagttcggtgtaggtcgttcgctccaagctgggctgtgtgcacgaaccccccgttcagcccgaccgctgcgccttatccggtaactatcgtcttgagtccaacccggtaagacacgacttatcgccactggcagcagccactggtaacaggattagcagagcgaggtatgtaggcggtgctacagagttcttgaagtggtggcctaactacggctacactagaaggacagtatttggtatctgcgctctgctgaagccagttaccttcggaaaaagagttggtagctcttgatccggcaaacaaaccaccgctggtagcggtggtttttttgtttgcaagcagcagattacgcgcagaaaaaaaggatctcaagaagatcctttgatcttttctacggggtctgacgctcagtggaacgaaaactcacgttaagggattttggtcatgagattatcaaaaaggatcttcacctagatccttttaaattaaaaatgaagttttaaatcaatctaaagtatatatgagtaaacttggtctgacagttaccaatgcttaatcagtgaggcacctatctcagcgatctgtctatttcgttcatccatagttgcctgactccccgtcgtgtagataactacgatacgggagggcttaccatctggccccagtgctgcaatgataccgcgagacccacgctcaccggctccagatttatcagcaataaaccagccagccggaagggccgagcgcagaagtggtcctgcaactttatccgcctccatccagtctattaattgttgccgggaagctagagtaagtagttcgccagttaatagtttgcgcaacgttgttgccattgctgcaggcatcgtggtgtcacgctcgtcgtttggtatggcttcattcagctccggttcccaacgatcaaggcgagttacatgatcccccatgttgtgcaaaaaagcggttagctccttcggtcctccgatcgttgtcagaagtaagttggccgcagtgttatcactcatggttatggcagcactgcataattctcttactgtcatgccatccgtaagatgcttttctgtgactggtgagtactcaaccaagtcattctgagaatagtgtatgcggcgaccgagttgctcttgcccggcgtcaatacgggataataccgcgccacatagcagaactttaaaagtgctcatcattggaaaacgttcttcggggcgaaaactctcaaggatcttaccgctgttgagatccagttcgatgtaacccactcgtgcacccaactgatcttcagcatcttttactttcaccagcgtttctgggtgagcaaaaacaggaaggcaaaatgccgcaaaaaagggaataagggcgacacggaaatgttgaatactcatactcttcctttttcaatattattgaagcatttatcagggttattgtctcatgagcggatacatatttgaatgtatttagaaaaataaacaaataggggttccgcgcacatttccccgaaaagtgccacctgaaattgtaaacgttaatattttgttaaaattcgcgttaaatttttgttaaatcagctcattttttaaccaataggccgaaatcggcaaaatcccttataaatcaaaagaatagaccgagatagggttgagtgttgttccagtttggaacaagagtccactattaaagaacgtggactccaacgtcaaagggcgaaaaaccgtctatcagggcgatggcccactacgtgaaccatcaccctaatcaagttttttggggtcgaggtgccgtaaagcactaaatcggaaccctaaagggagcccccgatttagagcttgacggggaaagccggcgaacgtggcgagaaaggaagggaagaaagcgaaaggagcgggcgctagggcgctggcaagtgtagcggtcacgctgcgcgtaaccaccacacccgccgcgcttaatgcgccgctacagggcgcgtcccattcgcca

SEQ ID NO: 65 - DNA, 8190 bp, artificial
  pF(G)r7(S)r3
atccggatatagttcctcctttcagcaaaaaacccctcaagacccgtttagaggccccaaggggttatgctagttattgctcagcggtggcagcagccaactcagcttcctttcgggctttgttagcagccggatctcagtggtggtggtggtggtgctcgagtgcggccgctcagaactgtgtcgggcgcatcaccgcatcaatgccgccatcaatgacgatctgcgcgccatgcacatagcttgcggccgggctcatcaaaaaggcgatgaccgacgccatctcggacggctcggcacggcggcccatgggaggaacgaacttggcaatggattcgccatagcgcgggtcctgcaggcccgcctgcagcaagggagtctcggttgcaccgggggcgatggtgttcaggcgcacgccagcctcgccccaggcggcggcgcgtttgcgcacagccaccgtcaaagcattcttgctgcccgcataggccagatttccgccctgctctcccgcatgttcgacaatggcgcgggccttggcttcctcgccggcttccagtgccagcgccagtgggttcttgtcaaaagccagatgcgcggaagccacggacgagatgacgacggctgcgggctgatggccttttttcagcgctggcaaaaaggcatccatcagctcggtcgcgccaaaataattgaccgaaaccacattgccaagcaccttggtctgcggtcccaggccggcgcacagcaccaggccgtccatgcccttgctgcacttcgccagtacatcggcaatcgcctgctttcgaccttcggccgtcgagagatcggcaatcacttccgcatcgcgtatatcgatgcctacgatctggtgaccggccgcctccaggaccttgcgcgtagcggcaccaatgccggtggcgcagccgcttatcacgatgatggacatgtatatctccttaagcttctagtcgcggtagaacgaccccatgtagcggatgtactcgtcctcggtgtggtttgccttccagtcgtggacggagtccttgttgcgctggccggcgatgacggagagctccttacccagcttctcaaaggcctcgtcaacgcactcctcgggggtgagggcgatcttcatgacggcctcgccctgcgggccgccggggaggttggacagcaggctgggggttagggtggtgccgagggtgatgacctcgacgtcgacgccggtgccctcgcactcgcaggccacggcctcggtcatcttgaggatgaaggccttgcccgcgccgtactggccgttccaggggctggagctgatgccggtcatcgacgagacgttgatcacggcgccgcggtcctgggcggcaaagatccgcatgtagtggtggaagcacttgaggaaggtcacgacgttgacgttgatcatggcctcgtgcttctcccagggggtgtcctggatcttaccgaagctgtgcaggcaggccacgtagctcatgaagcccatgtccaggccctcggtcgcggcgaagacggtctcggcagcgccgggctggctaaagtcggcgcgcacgaccttggtctccacgccgtaggtctcgcggatctcgcctgcgagcacgttcagcttctcctcgcgacggctgaccatgacgacgttcatgccgccggcggcgatcttctcgcagaacgccttgccgacgccctcggtcgcgcccaggatcaggccccactcaccgtacttctccctcaggttcatgtatatctcctttcacgaattctcagccgccttcttgaacttggcggcctcttccgaaccgccggtggcattgcccttcgagtaggaatgcgcgccggtgccggcaagagcgccgccctgcacgatgaggtattcgtcgcggatcggacggccctcgaagaagcactccaggatctcgcgggtgcccgccgcataacgcgcctgcgcggtcagcgtggtgccggagatgtgcggggtcatgccgttatagggcatcgtccgccaggggtggtccttcggcgccggctgcgggaaccacacgtcgccggcatagccggccagccggccggattcgagcgcacgtgccacggcatcgcggtcgcacagcttgccgcgggcggtgttgacgatgtaggcgccacgcttgaacagcttcagcgtctcgtcattgatcatgtgctcggtttcggggtgcagcgggcagttcagcgtcaccacgtcgcaaaccggatacatgtcctcgcgggtcgcgtgccaggtgaggttgagctccttctcgaccgattccggcaggcggtgacggccggtgtagtgcaggtgcacgtcgaacggcgccagacggcgcagcaccgcgagaccgatgcggccggcggccacggtgccgacatgcatcgcctcgaggtcgtaggcgtgggagacgcagtcggcgatgttccagccgcccttccgcgcccattcgtgcgagggcagatagttgcgcaccagcgacaggatcatcatcaccacatgctcggcgacgctgatcgagttgcagtaggtgacttccgccacggtgacgttgcggtcgatagccgactgaagatcgacgtggtcggaaccgatgccggcggtgagcgcgagcttcaggttcttggccttggcgatgcgctcgggcgtcagataggccggccagaagggctgggagatgacgacatccgcatcgaccagctcgcgctcgaacaccgagtcggggccgtccttgtcggaggtcacgaccagggtgtggccgttggattcgagatattcgcgcaggccgagctcgccggagacggagccgagcaactgcccgggcgtgaagtcgatggccttcggcgtcggcaagatctggccgcccggatagtggtcgatcttcggaagatcgtcgcgggcataggtcttcgggtagccgtcgaccggatcatcgtaaagaacgcacaggacctttgccatcatatgtatatctccttcttaaagttaaacaaaattatttctagaggggaattgttatccgctcacaattcccctatagtgagtcgtattaatttcgcgggatcgagatctcgatcctctacgccggacgcatcgtggccggcatcaccggcgccacaggtgcggttgctggcgcctatatcgccgacatcaccgatggggaagatcgggctcgccacttcgggctcatgagcgcttgtttcggcgtgggtatggtggcaggccccgtggccgggggactgttgggcgccatctccttgcatgcaccattccttgcggcggcggtgctcaacggcctcaacctactactgggctgcttcctaatgcaggagtcgcataagggagagcgtcgagatcccggacaccatcgaatggcgcaaaacctttcgcggtatggcatgatagcgcccggaagagagtcaattcagggtggtgaatgtgaaaccagtaacgttatacgatgtcgcagagtatgccggtgtctcttatcagaccgtttcccgcgtggtgaaccaggccagccacgtttctgcgaaaacgcgggaaaaagtggaagcggcgatggcggagctgaattacattcccaaccgcgtggcacaacaactggcgggcaaacagtcgttgctgattggcgttgccacctccagtctggccctgcacgcgccgtcgcaaattgtcgcggcgattaaatctcgcgccgatcaactgggtgccagcgtggtggtgtcgatggtagaacgaagcggcgtcgaagcctgtaaagcggcggtgcacaatcttctcgcgcaacgcgtcagtgggctgatcattaactatccgctggatgaccaggatgccattgctgtggaagctgcctgcactaatgttccggcgttatttcttgatgtctctgaccagacacccatcaacagtattattttctcccatgaagacggtacgcgactgggcgtggagcatctggtcgcattgggtcaccagcaaatcgcgctgttagcgggcccattaagttctgtctcggcgcgtctgcgtctggctggctggcataaatatctcactcgcaatcaaattcagccgatagcggaacgggaaggcgactggagtgccatgtccggttttcaacaaaccatgcaaatgctgaatgagggcatcgttcccactgcgatgctggttgccaacgatcagatggcgctgggcgcaatgcgcgccattaccgagtccgggctgcgcgttggtgcggatatctcggtagtgggatacgacgataccgaagacagctcatgttatatcccgccgttaaccaccatcaaacaggattttcgcctgctggggcaaaccagcgtggaccgcttgctgcaactctctcagggccaggcggtgaagggcaatcagctgttgcccgtctcactggtgaaaagaaaaaccaccctggcgcccaatacgcaaaccgcctctccccgcgcgttggccgattcattaatgcagctggcacgacaggtttcccgactggaaagcgggcagtgagcgcaacgcaattaatgtaagttagctcactcattaggcaccgggatctcgaccgatgcccttgagagccttcaacccagtcagctccttccggtgggcgcggggcatgactatcgtcgccgcacttatgactgtcttctttatcatgcaactcgtaggacaggtgccggcagcgctctgggtcattttcggcgaggaccgctttcgctggagcgcgacgatgatcggcctgtcgcttgcggtattcggaatcttgcacgccctcgctcaagccttcgtcactggtcccgccaccaaacgtttcggcgagaagcaggccattatcgccggcatggcggccccacgggtgcgcatgatcgtgctcctgtcgttgaggacccggctaggctggcggggttgccttactggttagcagaatgaatcaccgatacgcgagcgaacgtgaagcgactgctgctgcaaaacgtctgcgacctgagcaacaacatgaatggtcttcggtttccgtgtttcgtaaagtctggaaacgcggaagtcagcgccctgcaccattatgttccggatctgcatcgcaggatgctgctggctaccctgtggaacacctacatctgtattaacgaagcgctggcattgaccctgagtgatttttctctggtcccgccgcatccataccgccagttgtttaccctcacaacgttccagtaaccgggcatgttcatcatcagtaacccgtatcgtgagcatcctctctcgtttcatcggtatcattacccccatgaacagaaatcccccttacacggaggcatcagtgaccaaacaggaaaaaaccgcccttaacatggcccgctttatcagaagccagacattaacgcttctggagaaactcaacgagctggacgcggatgaacaggcagacatctgtgaatcgcttcacgaccacgctgatgagctttaccgcagctgcctcgcgcgtttcggtgatgacggtgaaaacctctgacacatgcagctcccggagacggtcacagcttgtctgtaagcggatgccgggagcagacaagcccgtcagggcgcgtcagcgggtgttggcgggtgtcggggcgcagccatgacccagtcacgtagcgatagcggagtgtatactggcttaactatgcggcatcagagcagattgtactgagagtgcaccatatatgcggtgtgaaataccgcacagatgcgtaaggagaaaataccgcatcaggcgctcttccgcttcctcgctcactgactcgctgcgctcggtcgttcggctgcggcgagcggtatcagctcactcaaaggcggtaatacggttatccacagaatcaggggataacgcaggaaagaacatgtgagcaaaaggccagcaaaaggccaggaaccgtaaaaaggccgcgttgctggcgtttttccataggctccgcccccctgacgagcatcacaaaaatcgacgctcaagtcagaggtggcgaaacccgacaggactataaagataccaggcgtttccccctggaagctccctcgtgcgctctcctgttccgaccctgccgcttaccggatacctgtccgcctttctcccttcgggaagcgtggcgctttctcatagctcacgctgtaggtatctcagttcggtgtaggtcgttcgctccaagctgggctgtgtgcacgaaccccccgttcagcccgaccgctgcgccttatccggtaactatcgtcttgagtccaacccggtaagacacgacttatcgccactggcagcagccactggtaacaggattagcagagcgaggtatgtaggcggtgctacagagttcttgaagtggtggcctaactacggctacactagaaggacagtatttggtatctgcgctctgctgaagccagttaccttcggaaaaagagttggtagctcttgatccggcaaacaaaccaccgctggtagcggtggtttttttgtttgcaagcagcagattacgcgcagaaaaaaaggatctcaagaagatcctttgatcttttctacggggtctgacgctcagtggaacgaaaactcacgttaagggattttggtcatgagattatcaaaaaggatcttcacctagatccttttaaattaaaaatgaagttttaaatcaatctaaagtatatatgagtaaacttggtctgacagttaccaatgcttaatcagtgaggcacctatctcagcgatctgtctatttcgttcatccatagttgcctgactccccgtcgtgtagataactacgatacgggagggcttaccatctggccccagtgctgcaatgataccgcgagacccacgctcaccggctccagatttatcagcaataaaccagccagccggaagggccgagcgcagaagtggtcctgcaactttatccgcctccatccagtctattaattgttgccgggaagctagagtaagtagttcgccagttaatagtttgcgcaacgttgttgccattgctgcaggcatcgtggtgtcacgctcgtcgtttggtatggcttcattcagctccggttcccaacgatcaaggcgagttacatgatcccccatgttgtgcaaaaaagcggttagctccttcggtcctccgatcgttgtcagaagtaagttggccgcagtgttatcactcatggttatggcagcactgcataattctcttactgtcatgccatccgtaagatgcttttctgtgactggtgagtactcaaccaagtcattctgagaatagtgtatgcggcgaccgagttgctcttgcccggcgtcaatacgggataataccgcgccacatagcagaactttaaaagtgctcatcattggaaaacgttcttcggggcgaaaactctcaaggatcttaccgctgttgagatccagttcgatgtaacccactcgtgcacccaactgatcttcagcatcttttactttcaccagcgtttctgggtgagcaaaaacaggaaggcaaaatgccgcaaaaaagggaataagggcgacacggaaatgttgaatactcatactcttcctttttcaatattattgaagcatttatcagggttattgtctcatgagcggatacatatttgaatgtatttagaaaaataaacaaataggggttccgcgcacatttccccgaaaagtgccacctgaaattgtaaacgttaatattttgttaaaattcgcgttaaatttttgttaaatcagctcattttttaaccaataggccgaaatcggcaaaatcccttataaatcaaaagaatagaccgagatagggttgagtgttgttccagtttggaacaagagtccactattaaagaacgtggactccaacgtcaaagggcgaaaaaccgtctatcagggcgatggcccactacgtgaaccatcaccctaatcaagttttttggggtcgaggtgccgtaaagcactaaatcggaaccctaaagggagcccccgatttagagcttgacggggaaagccggcgaacgtggcgagaaaggaagggaagaaagcgaaaggagcgggcgctagggcgctggcaagtgtagcggtcacgctgcgcgtaaccaccacacccgccgcgcttaatgcgccgctacagggcgcgtcccattcgcca

SEQ ID NO: 66 - DNA, 7910 bp, artificial
  p3T7(A)rG
atccggatatagttcctcctttcagcaaaaaacccctcaagacccgtttagaggccccaaggggttatgctagttattgctcagcggtggcagcagccaactcagcttcctttcgggctttgttagcagccggatctcagtggtggtggtggtggtgctcgagttaaccgcggcctgcctggaatgaaggatattgtgtcataccgccgtccgcgaataacgtgatgcctgtgacgtagctggcttccttcgaagcaagccaggctgctactgcggcgatctcctccggttcgccgatatatcccattggaatcatgctttctacatcagctttctgtttagggtcagcgaatttttcagcattgattggcgtgttgatcgcacctggcccaatattattgacgcgaatgcccttcggcgcgtattccaacgctaatgtttctgtcatcagctttatcccgcctttacttgccgcatagtggacaaataacggccaaggaatcacttcgtgcacactggacatgttaatgacatttcccttgatatcgttttctacgaaatatttaatcgcttcacggcttcctaaaaaggcacccgttaagttcgtgccgatgactttatcccaatccttgagcggcatttcgtgagatggcacaggattttcaagaccggcattattaatcataatatcgagtgtgccgaactccttaattgccgtttgcacgatattttttacatcttcctctttcgtgacatctccttggacgacaacagcttcaccgcccgccttgatgacctcttcttttacctcgttcggatcttgtttattactataatagttgataaccacttttgcctgctccttgccgaagcgaatggccatcgcctttccgagccctgaagcagctcctgtaatagcgacgacttttccttttaaatccggatacatgtatatctccttgcggccgcctagtcgcggtagaacgaccccatgtagcggatgtactcgtcctcggtgtggtttgccttccagtcgtggacggagtccttgttgcgctggccggcgatgacggagagctccttacccagcttctcaaaggcctcgtcaacgcactcctcgggggtgagggcgatcttcatgacggcctcgccctgcgggccgccggggaggttggacagcaggctgggggttagggtggtgccgagggtgatgacctcgacgtcgacgccggtgccctcgcactcgcaggccacggcctcggtcatcttgaggatgaaggccttgcccgcgccgtactggccgttccaggggctggagctgatgccggtcatcgacgagacgttgatcacggcgccgcggtcctgggcggcaaagatccgcatgtagtggtggaagcacttgaggaaggtcacgacgttgacgttgatcatggcctcgtgcttctcccagggggtgtcctggatcttaccgaagctgtgcaggcaggccacgtagctcatgaagcccatgtccaggccctcggtcgcggcgaagacggtctcggcagcgccgggctggctaaagtcggcgcgcacgaccttggtctccacgccgtaggtctcgcggatctcgcctgcgagcacgttcagcttctcctcgcgacgggcgaccatgacgacgttcatgccgccggcggcgatcttctcgcagaacgccttgccgacgccctcggtcgcgcccaggatcaggccccactcaccgtacttctccctcaggttcatatgtatatctccttcttatacttaactaatatactaagatggggaattgttatccgctcacaattcccctatagtgagtcgtattaatttcgattatgcggccgtgtacaatacgattactttctgttcgacttaagcattataagcttgtcgacggagctcgaattctcagaactgtgtcgggcgcatcaccgcatcaatgccgccatcaatgacgatctgcgcgccatgcacatagcttgcggccgggctcatcaaaaaggcgatgaccgacgccatctcggacggctcggcacggcggcccatgggaggaacgaacttggcaatggattcgccatagcgcgggtcctgcaggcccgcctgcagcaagggagtctcggttgcaccgggggcgatggtgttcaggcgcacgccagcctcgccccaggcggcggcgcgtttgcgcacagccaccgtcaaagcattcttgctgcccgcataggccagatttccgccctgctctcccgcatgttcgacaatggcgcgggccttggcttcctcgccggcttccagtgccagcgccagtgggttcttgtcaaaagccagatgcgcggaagccacggacgagatgacgacggctgcgggctgatggccttttttcagcgctggcaaaaaggcatccatcagctcggtcgcgccaaaataattgaccgaaaccacattgccaagcaccttggtctgcggtcccaggccggcgcacagcaccaggccgtccatgcccttgctgcacttcgccagtacatcggcaatcgcctgctttcgaccttcggccgtcgagagatcggcaatcacttccgcatcgcgtatatcgatgcctacgatctggtgaccggccgcctccaggaccttgcgcgtagccgcaccaatgccggtggcgcagccgcttatcacgatgatggacatcatatgtatatctccttcttaaagttaaacaaaattatttctagaggggaattgttatccgctcacaattcccctatagtgagtcgtattaatttcgcgggatcgagatctcgatcctctacgccggacgcatcgtggccggcatcaccggcgccacaggtgcggttgctggcgcctatatcgccgacatcaccgatggggaagatcgggctcgccacttcgggctcatgagcgcttgtttcggcgtgggtatggtggcaggccccgtggccgggggactgttgggcgccatctccttgcatgcaccattccttgcggcggcggtgctcaacggcctcaacctactactgggctgcttcctaatgcaggagtcgcataagggagagcgtcgagatcccggacaccatcgaatggcgcaaaacctttcgcggtatggcatgatagcgcccggaagagagtcaattcagggtggtgaatgtgaaaccagtaacgttatacgatgtcgcagagtatgccggtgtctcttatcagaccgtttcccgcgtggtgaaccaggccagccacgtttctgcgaaaacgcgggaaaaagtggaagcggcgatggcggagctgaattacattcccaaccgcgtggcacaacaactggcgggcaaacagtcgttgctgattggcgttgccacctccagtctggccctgcacgcgccgtcgcaaattgtcgcggcgattaaatctcgcgccgatcaactgggtgccagcgtggtggtgtcgatggtagaacgaagcggcgtcgaagcctgtaaagcggcggtgcacaatcttctcgcgcaacgcgtcagtgggctgatcattaactatccgctggatgaccaggatgccattgctgtggaagctgcctgcactaatgttccggcgttatttcttgatgtctctgaccagacacccatcaacagtattattttctcccatgaagacggtacgcgactgggcgtggagcatctggtcgcattgggtcaccagcaaatcgcgctgttagcgggcccattaagttctgtctcggcgcgtctgcgtctggctggctggcataaatatctcactcgcaatcaaattcagccgatagcggaacgggaaggcgactggagtgccatgtccggttttcaacaaaccatgcaaatgctgaatgagggcatcgttcccactgcgatgctggttgccaacgatcagatggcgctgggcgcaatgcgcgccattaccgagtccgggctgcgcgttggtgcggatatctcggtagtgggatacgacgataccgaagacagctcatgttatatcccgccgttaaccaccatcaaacaggattttcgcctgctggggcaaaccagcgtggaccgcttgctgcaactctctcagggccaggcggtgaagggcaatcagctgttgcccgtctcactggtgaaaagaaaaaccaccctggcgcccaatacgcaaaccgcctctccccgcgcgttggccgattcattaatgcagctggcacgacaggtttcccgactggaaagcgggcagtgagcgcaacgcaattaatgtaagttagctcactcattaggcaccgggatctcgaccgatgcccttgagagccttcaacccagtcagctccttccggtgggcgcggggcatgactatcgtcgccgcacttatgactgtcttctttatcatgcaactcgtaggacaggtgccggcagcgctctgggtcattttcggcgaggaccgctttcgctggagcgcgacgatgatcggcctgtcgcttgcggtattcggaatcttgcacgccctcgctcaagccttcgtcactggtcccgccaccaaacgtttcggcgagaagcaggccattatcgccggcatggcggccccacgggtgcgcatgatcgtgctcctgtcgttgaggacccggctaggctggcggggttgccttactggttagcagaatgaatcaccgatacgcgagcgaacgtgaagcgactgctgctgcaaaacgtctgcgacctgagcaacaacatgaatggtcttcggtttccgtgtttcgtaaagtctggaaacgcggaagtcagcgccctgcaccattatgttccggatctgcatcgcaggatgctgctggctaccctgtggaacacctacatctgtattaacgaagcgctggcattgaccctgagtgatttttctctggtcccgccgcatccataccgccagttgtttaccctcacaacgttccagtaaccgggcatgttcatcatcagtaacccgtatcgtgagcatcctctctcgtttcatcggtatcattacccccatgaacagaaatcccccttacacggaggcatcagtgaccaaacaggaaaaaaccgcccttaacatggcccgctttatcagaagccagacattaacgcttctggagaaactcaacgagctggacgcggatgaacaggcagacatctgtgaatcgcttcacgaccacgctgatgagctttaccgcagctgcctcgcgcgtttcggtgatgacggtgaaaacctctgacacatgcagctcccggagacggtcacagcttgtctgtaagcggatgccgggagcagacaagcccgtcagggcgcgtcagcgggtgttggcgggtgtcggggcgcagccatgacccagtcacgtagcgatagcggagtgtatactggcttaactatgcggcatcagagcagattgtactgagagtgcaccatatatgcggtgtgaaataccgcacagatgcgtaaggagaaaataccgcatcaggcgctcttccgcttcctcgctcactgactcgctgcgctcggtcgttcggctgcggcgagcggtatcagctcactcaaaggcggtaatacggttatccacagaatcaggggataacgcaggaaagaacatgtgagcaaaaggccagcaaaaggccaggaaccgtaaaaaggccgcgttgctggcgtttttccataggctccgcccccctgacgagcatcacaaaaatcgacgctcaagtcagaggtggcgaaacccgacaggactataaagataccaggcgtttccccctggaagctccctcgtgcgctctcctgttccgaccctgccgcttaccggatacctgtccgcctttctcccttcgggaagcgtggcgctttctcatagctcacgctgtaggtatctcagttcggtgtaggtcgttcgctccaagctgggctgtgtgcacgaaccccccgttcagcccgaccgctgcgccttatccggtaactatcgtcttgagtccaacccggtaagacacgacttatcgccactggcagcagccactggtaacaggattagcagagcgaggtatgtaggcggtgctacagagttcttgaagtggtggcctaactacggctacactagaaggacagtatttggtatctgcgctctgctgaagccagttaccttcggaaaaagagttggtagctcttgatccggcaaacaaaccaccgctggtagcggtggtttttttgtttgcaagcagcagattacgcgcagaaaaaaaggatctcaagaagatcctttgatcttttctacggggtctgacgctcagtggaacgaaaactcacgttaagggattttggtcatgagattatcaaaaaggatcttcacctagatccttttaaattaaaaatgaagttttaaatcaatctaaagtatatatgagtaaacttggtctgacagttaccaatgcttaatcagtgaggcacctatctcagcgatctgtctatttcgttcatccatagttgcctgactccccgtcgtgtagataactacgatacgggagggcttaccatctggccccagtgctgcaatgataccgcgagacccacgctcaccggctccagatttatcagcaataaaccagccagccggaagggccgagcgcagaagtggtcctgcaactttatccgcctccatccagtctattaattgttgccgggaagctagagtaagtagttcgccagttaatagtttgcgcaacgttgttgccattgctgcaggcatcgtggtgtcacgctcgtcgtttggtatggcttcattcagctccggttcccaacgatcaaggcgagttacatgatcccccatgttgtgcaaaaaagcggttagctccttcggtcctccgatcgttgtcagaagtaagttggccgcagtgttatcactcatggttatggcagcactgcataattctcttactgtcatgccatccgtaagatgcttttctgtgactggtgagtactcaaccaagtcattctgagaatagtgtatgcggcgaccgagttgctcttgcccggcgtcaatacgggataataccgcgccacatagcagaactttaaaagtgctcatcattggaaaacgttcttcggggcgaaaactctcaaggatcttaccgctgttgagatccagttcgatgtaacccactcgtgcacccaactgatcttcagcatcttttactttcaccagcgtttctgggtgagcaaaaacaggaaggcaaaatgccgcaaaaaagggaataagggcgacacggaaatgttgaatactcatactcttcctttttcaatattattgaagcatttatcagggttattgtctcatgagcggatacatatttgaatgtatttagaaaaataaacaaataggggttccgcgcacatttccccgaaaagtgccacctgaaattgtaaacgttaatattttgttaaaattcgcgttaaatttttgttaaatcagctcattttttaaccaataggccgaaatcggcaaaatcccttataaatcaaaagaatagaccgagatagggttgagtgttgttccagtttggaacaagagtccactattaaagaacgtggactccaacgtcaaagggcgaaaaaccgtctatcagggcgatggcccactacgtgaaccatcaccctaatcaagttttttggggtcgaggtgccgtaaagcactaaatcggaaccctaaagggagcccccgatttagagcttgacggggaaagccggcgaacgtggcgagaaaggaagggaagaaagcgaaaggagcgggcgctagggcgctggcaagtgtagcggtcacgctgcgcgtaaccaccacacccgccgcgcttaatgcgccgctacagggcgcgtcccattcgcca

SEQ ID NO: 67 - DNA, 7891 bp, artificial
  p7(A)T3rG
atccggatatagttcctcctttcagcaaaaaacccctcaagacccgtttagaggccccaaggggttatgctagttattgctcagcggtggcagcagccaactcagcttcctttcgggctttgttagcagccggatctcagtggtggtggtggtggtgctcgagttaaccgcggcctgcctggaatgaaggatattgtgtcataccgccgtccgcgaataacgtgatgcctgtgacgtagctggcttccttcgaagcaagccaggctgctactgcggcgatctcctccggttcgccgatatatcccattggaatcatgctttctacatcagctttctgtttagggtcagcgaatttttcagcattgattggcgtgttgatcgcacctggcccaatattattgacgcgaatgcccttcggcgcgtattccaacgctaatgtttctgtcatcagctttatcccgcctttacttgccgcatagtggacaaataacggccaaggaatcacttcgtgcacactggacatgttaatgacatttcccttgatatcgttttctacgaaatatttaatcgcttcacggcttcctaaaaaggcacccgttaagttcgtgccgatgactttatcccaatccttgagcggcatttcgtgagatggcacaggattttcaagaccggcattattaatcataatatcgagtgtgccgaactccttaattgccgtttgcacgatattttttacatcttcctctttcgtgacatctccttggacgacaacagcttcaccgcccgccttgatgacctcttcttttacctcgttcggatcttgtttattactataatagttgataaccacttttgcctgctccttgccgaagcgaatggccatcgcctttccgagccctgaagcagctcctgtaatagcgacgacttttccttttaaatccggatacatgtatatctccttgcggccgctcagaactgtgtcgggcgcatcaccgcatcaatgccgccatcaatgacgatctgcgcgccatgcacatagcttgcggccgggctcatcaaaaaggcgatgaccgacgccatctcggacggctcggcacggcggcccatgggaggaacgaacttggcaatggattcgccatagcgcgggtcctgcaggcccgcctgcagcaagggagtctcggttgcaccgggggcgatggtgttcaggcgcacgccagcctcgccccaggcggcggcgcgtttgcgcacagccaccgtcaaagcattcttgctgcccgcataggccagatttccgccctgctctcccgcatgttcgacaatggcgcgggccttggcttcctcgccggcttccagtgccagcgccagtgggttcttgtcaaaagccagatgcgcggaagccacggacgagatgacgacggctgcgggctgatggccttttttcagcgctggcaaaaaggcatccatcagctcggtcgcgccaaaataattgaccgaaaccacattgccaagcaccttggtctgcggtcccaggccggcgcacagcaccaggccgtccatgcccttgctgcacttcgccagtacatcggcaatcgcctgctttcgaccttcggccgtcgagagatcggcaatcacttccgcatcgcgtatatcgatgcctacgatctggtgaccggccgcctccaggaccttgcgcgtagcggcaccaatgccggtggcgcagccgcttatcacgatgatggacatcatatgtatatctccttcttatacttaactaatatactaagatggggaattgttatccgctcacaattcccctatagtgagtcgtattaatttcgattatgcggccgtgtacaatacgattactttctgttcgacttaagcattataagcttctagtcgcggtagaacgaccccatgtagcggatgtactcgtcctcggtgtggtttgccttccagtcgtggacggagtccttgttgcgctggccggcgatgacggagagctccttacccagcttctcaaaggcctcgtcaacgcactcctcgggggtgagggcgatcttcatgacggcctcgccctgcgggccgccggggaggttggacagcaggctgggggttagggtggtgccgagggtgatgacctcgacgtcgacgccggtgccctcgcactcgcaggccacggcctcggtcatcttgaggatgaaggccttgcccgcgccgtactggccgttccaggggctggagctgatgccggtcatcgacgagacgttgatcacggcgccgcggtcctgggcggcaaagatccgcatgtagtggtggaagcacttgaggaaggtcacgacgttgacgttgatcatggcctcgtgcttctcccagggggtgtcctggatcttaccgaagctgtgcaggcaggccacgtagctcatgaagcccatgtccaggccctcggtcgcggcgaagacggtctcggcagcgccgggctggctaaagtcggcgcgcacgaccttggtctccacgccgtaggtctcgcggatctcgcctgcgagcacgttcagcttctcctcgcgacgggcgaccatgacgacgttcatgccgccggcggcgatcttctcgcagaacgccttgccgacgccctcggtcgcgcccaggatcaggccccactcaccgtacttctccctcaggttcatatgtatatctccttcttaaagttaaacaaaattatttctagaggggaattgttatccgctcacaattcccctatagtgagtcgtattaatttcgcgggatcgagatctcgatcctctacgccggacgcatcgtggccggcatcaccggcgccacaggtgcggttgctggcgcctatatcgccgacatcaccgatggggaagatcgggctcgccacttcgggctcatgagcgcttgtttcggcgtgggtatggtggcaggccccgtggccgggggactgttgggcgccatctccttgcatgcaccattccttgcggcggcggtgctcaacggcctcaacctactactgggctgcttcctaatgcaggagtcgcataagggagagcgtcgagatcccggacaccatcgaatggcgcaaaacctttcgcggtatggcatgatagcgcccggaagagagtcaattcagggtggtgaatgtgaaaccagtaacgttatacgatgtcgcagagtatgccggtgtctcttatcagaccgtttcccgcgtggtgaaccaggccagccacgtttctgcgaaaacgcgggaaaaagtggaagcggcgatggcggagctgaattacattcccaaccgcgtggcacaacaactggcgggcaaacagtcgttgctgattggcgttgccacctccagtctggccctgcacgcgccgtcgcaaattgtcgcggcgattaaatctcgcgccgatcaactgggtgccagcgtggtggtgtcgatggtagaacgaagcggcgtcgaagcctgtaaagcggcggtgcacaatcttctcgcgcaacgcgtcagtgggctgatcattaactatccgctggatgaccaggatgccattgctgtggaagctgcctgcactaatgttccggcgttatttcttgatgtctctgaccagacacccatcaacagtattattttctcccatgaagacggtacgcgactgggcgtggagcatctggtcgcattgggtcaccagcaaatcgcgctgttagcgggcccattaagttctgtctcggcgcgtctgcgtctggctggctggcataaatatctcactcgcaatcaaattcagccgatagcggaacgggaaggcgactggagtgccatgtccggttttcaacaaaccatgcaaatgctgaatgagggcatcgttcccactgcgatgctggttgccaacgatcagatggcgctgggcgcaatgcgcgccattaccgagtccgggctgcgcgttggtgcggatatctcggtagtgggatacgacgataccgaagacagctcatgttatatcccgccgttaaccaccatcaaacaggattttcgcctgctggggcaaaccagcgtggaccgcttgctgcaactctctcagggccaggcggtgaagggcaatcagctgttgcccgtctcactggtgaaaagaaaaaccaccctggcgcccaatacgcaaaccgcctctccccgcgcgttggccgattcattaatgcagctggcacgacaggtttcccgactggaaagcgggcagtgagcgcaacgcaattaatgtaagttagctcactcattaggcaccgggatctcgaccgatgcccttgagagccttcaacccagtcagctccttccggtgggcgcggggcatgactatcgtcgccgcacttatgactgtcttctttatcatgcaactcgtaggacaggtgccggcagcgctctgggtcattttcggcgaggaccgctttcgctggagcgcgacgatgatcggcctgtcgcttgcggtattcggaatcttgcacgccctcgctcaagccttcgtcactggtcccgccaccaaacgtttcggcgagaagcaggccattatcgccggcatggcggccccacgggtgcgcatgatcgtgctcctgtcgttgaggacccggctaggctggcggggttgccttactggttagcagaatgaatcaccgatacgcgagcgaacgtgaagcgactgctgctgcaaaacgtctgcgacctgagcaacaacatgaatggtcttcggtttccgtgtttcgtaaagtctggaaacgcggaagtcagcgccctgcaccattatgttccggatctgcatcgcaggatgctgctggctaccctgtggaacacctacatctgtattaacgaagcgctggcattgaccctgagtgatttttctctggtcccgccgcatccataccgccagttgtttaccctcacaacgttccagtaaccgggcatgttcatcatcagtaacccgtatcgtgagcatcctctctcgtttcatcggtatcattacccccatgaacagaaatcccccttacacggaggcatcagtgaccaaacaggaaaaaaccgcccttaacatggcccgctttatcagaagccagacattaacgcttctggagaaactcaacgagctggacgcggatgaacaggcagacatctgtgaatcgcttcacgaccacgctgatgagctttaccgcagctgcctcgcgcgtttcggtgatgacggtgaaaacctctgacacatgcagctcccggagacggtcacagcttgtctgtaagcggatgccgggagcagacaagcccgtcagggcgcgtcagcgggtgttggcgggtgtcggggcgcagccatgacccagtcacgtagcgatagcggagtgtatactggcttaactatgcggcatcagagcagattgtactgagagtgcaccatatatgcggtgtgaaataccgcacagatgcgtaaggagaaaataccgcatcaggcgctcttccgcttcctcgctcactgactcgctgcgctcggtcgttcggctgcggcgagcggtatcagctcactcaaaggcggtaatacggttatccacagaatcaggggataacgcaggaaagaacatgtgagcaaaaggccagcaaaaggccaggaaccgtaaaaaggccgcgttgctggcgtttttccataggctccgcccccctgacgagcatcacaaaaatcgacgctcaagtcagaggtggcgaaacccgacaggactataaagataccaggcgtttccccctggaagctccctcgtgcgctctcctgttccgaccctgccgcttaccggatacctgtccgcctttctcccttcgggaagcgtggcgctttctcatagctcacgctgtaggtatctcagttcggtgtaggtcgttcgctccaagctgggctgtgtgcacgaaccccccgttcagcccgaccgctgcgccttatccggtaactatcgtcttgagtccaacccggtaagacacgacttatcgccactggcagcagccactggtaacaggattagcagagcgaggtatgtaggcggtgctacagagttcttgaagtggtggcctaactacggctacactagaaggacagtatttggtatctgcgctctgctgaagccagttaccttcggaaaaagagttggtagctcttgatccggcaaacaaaccaccgctggtagcggtggtttttttgtttgcaagcagcagattacgcgcagaaaaaaaggatctcaagaagatcctttgatcttttctacggggtctgacgctcagtggaacgaaaactcacgttaagggattttggtcatgagattatcaaaaaggatcttcacctagatccttttaaattaaaaatgaagttttaaatcaatctaaagtatatatgagtaaacttggtctgacagttaccaatgcttaatcagtgaggcacctatctcagcgatctgtctatttcgttcatccatagttgcctgactccccgtcgtgtagataactacgatacgggagggcttaccatctggccccagtgctgcaatgataccgcgagacccacgctcaccggctccagatttatcagcaataaaccagccagccggaagggccgagcgcagaagtggtcctgcaactttatccgcctccatccagtctattaattgttgccgggaagctagagtaagtagttcgccagttaatagtttgcgcaacgttgttgccattgctgcaggcatcgtggtgtcacgctcgtcgtttggtatggcttcattcagctccggttcccaacgatcaaggcgagttacatgatcccccatgttgtgcaaaaaagcggttagctccttcggtcctccgatcgttgtcagaagtaagttggccgcagtgttatcactcatggttatggcagcactgcataattctcttactgtcatgccatccgtaagatgcttttctgtgactggtgagtactcaaccaagtcattctgagaatagtgtatgcggcgaccgagttgctcttgcccggcgtcaatacgggataataccgcgccacatagcagaactttaaaagtgctcatcattggaaaacgttcttcggggcgaaaactctcaaggatcttaccgctgttgagatccagttcgatgtaacccactcgtgcacccaactgatcttcagcatcttttactttcaccagcgtttctgggtgagcaaaaacaggaaggcaaaatgccgcaaaaaagggaataagggcgacacggaaatgttgaatactcatactcttcctttttcaatattattgaagcatttatcagggttattgtctcatgagcggatacatatttgaatgtatttagaaaaataaacaaataggggttccgcgcacatttccccgaaaagtgccacctgaaattgtaaacgttaatattttgttaaaattcgcgttaaatttttgttaaatcagctcattttttaaccaataggccgaaatcggcaaaatcccttataaatcaaaagaatagaccgagatagggttgagtgttgttccagtttggaacaagagtccactattaaagaacgtggactccaacgtcaaagggcgaaaaaccgtctatcagggcgatggcccactacgtgaaccatcaccctaatcaagttttttggggtcgaggtgccgtaaagcactaaatcggaaccctaaagggagcccccgatttagagcttgacggggaaagccggcgaacgtggcgagaaaggaagggaagaaagcgaaaggagcgggcgctagggcgctggcaagtgtagcggtcacgctgcgcgtaaccaccacacccgccgcgcttaatgcgccgctacagggcgcgtcccattcgcca

SEQ ID NO: 68 - DNA, 7404 bp, artificial
  pF(G)r7(A)
atccggatatagttcctcctttcagcaaaaaacccctcaagacccgtttagaggccccaaggggttatgctagttattgctcagcggtggcagcagccaactcagcttcctttcgggctttgttagcagccggatctcagtggtggtggtggtggtgctcgagtgcggccgcaagcttctagtcgcggtagaacgaccccatgtagcggatgtactcgtcctcggtgtggtttgccttccagtcgtggacggagtccttgttgcgctggccggcgatgacggagagctccttacccagcttctcaaaggcctcgtcaacgcactcctcgggggtgagggcgatcttcatgacggcctcgccctgcgggccgccggggaggttggacagcaggctgggggttagggtggtgccgagggtgatgacctcgacgtcgacgccggtgccctcgcactcgcaggccacggcctcggtcatcttgaggatgaaggccttgcccgcgccgtactggccgttccaggggctggagctgatgccggtcatcgacgagacgttgatcacggcgccgcggtcctgggcggcaaagatccgcatgtagtggtggaagcacttgaggaaggtcacgacgttgacgttgatcatggcctcgtgcttctcccagggggtgtcctggatcttaccgaagctgtgcaggcaggccacgtagctcatgaagcccatgtccaggccctcggtcgcggcgaagacggtctcggcagcgccgggctggctaaagtcggcgcgcacgaccttggtctccacgccgtaggtctcgcggatctcgcctgcgagcacgttcagcttctcctcgcgacgggcgaccatgacgacgttcatgccgccggcggcgatcttctcgcagaacgccttgccgacgccctcggtcgcgcccaggatcaggccccactcaccgtacttctccctcaggttcatgtatatctcctttcacgaattctcagccgccttcttgaacttggcggcctcttccgaaccgccggtggcattgcccttcgagtaggaatgcgcgccggtgccggcaagagcgccgccctgcacgatgaggtattcgtcgcggatcggacggccctcgaagaagcactccaggatctcgcgggtgcccgccgcataacgcgcctgcgcggtcagcgtggtgccggagatgtgcggggtcatgccgttatagggcatcgtccgccaggggtggtccttcggcgccggctgcgggaaccacacgtcgccggcatagccggccagccggccggattcgagcgcacgtgccacggcatcgcggtcgcacagcttgccgcgggcggtgttgacgatgtaggcgccacgcttgaacagcttcagcgtctcgtcattgatcatgtgctcggtttcggggtgcagcgggcagttcagcgtcaccacgtcgcaaaccggatacatgtcctcgcgggtcgcgtgccaggtgaggttgagctccttctcgaccgattccggcaggcggtgacggccggtgtagtgcaggtgcacgtcgaacggcgccagacggcgcagcaccgcgagaccgatgcggccggcggccacggtgccgacatgcatcgcctcgaggtcgtaggcgtgggagacgcagtcggcgatgttccagccgcccttccgcgcccattcgtgcgagggcagatagttgcgcaccagcgacaggatcatcatcaccacatgctcggcgacgctgatcgagttgcagtaggtgacttccgccacggtgacgttgcggtcgatagccgactgaagatcgacgtggtcggaaccgatgccggcggtgagcgcgagcttcaggttcttggccttggcgatgcgctcgggcgtcagataggccggccagaagggctgggagatgacgacatccgcatcgaccagctcgcgctcgaacaccgagtcggggccgtccttgtcggaggtcacgaccagggtgtggccgttggattcgagatattcgcgcaggccgagctcgccggagacggagccgagcaactgcccgggcgtgaagtcgatggccttcggcgtcggcaagatctggccgcccggatagtggtcgatcttcggaagatcgtcgcgggcataggtcttcgggtagccgtcgaccggatcatcgtaaagaacgcacaggacctttgccatcatatgtatatctccttcttaaagttaaacaaaattatttctagaggggaattgttatccgctcacaattcccctatagtgagtcgtattaatttcgcgggatcgagatctcgatcctctacgccggacgcatcgtggccggcatcaccggcgccacaggtgcggttgctggcgcctatatcgccgacatcaccgatggggaagatcgggctcgccacttcgggctcatgagcgcttgtttcggcgtgggtatggtggcaggccccgtggccgggggactgttgggcgccatctccttgcatgcaccattccttgcggcggcggtgctcaacggcctcaacctactactgggctgcttcctaatgcaggagtcgcataagggagagcgtcgagatcccggacaccatcgaatggcgcaaaacctttcgcggtatggcatgatagcgcccggaagagagtcaattcagggtggtgaatgtgaaaccagtaacgttatacgatgtcgcagagtatgccggtgtctcttatcagaccgtttcccgcgtggtgaaccaggccagccacgtttctgcgaaaacgcgggaaaaagtggaagcggcgatggcggagctgaattacattcccaaccgcgtggcacaacaactggcgggcaaacagtcgttgctgattggcgttgccacctccagtctggccctgcacgcgccgtcgcaaattgtcgcggcgattaaatctcgcgccgatcaactgggtgccagcgtggtggtgtcgatggtagaacgaagcggcgtcgaagcctgtaaagcggcggtgcacaatcttctcgcgcaacgcgtcagtgggctgatcattaactatccgctggatgaccaggatgccattgctgtggaagctgcctgcactaatgttccggcgttatttcttgatgtctctgaccagacacccatcaacagtattattttctcccatgaagacggtacgcgactgggcgtggagcatctggtcgcattgggtcaccagcaaatcgcgctgttagcgggcccattaagttctgtctcggcgcgtctgcgtctggctggctggcataaatatctcactcgcaatcaaattcagccgatagcggaacgggaaggcgactggagtgccatgtccggttttcaacaaaccatgcaaatgctgaatgagggcatcgttcccactgcgatgctggttgccaacgatcagatggcgctgggcgcaatgcgcgccattaccgagtccgggctgcgcgttggtgcggatatctcggtagtgggatacgacgataccgaagacagctcatgttatatcccgccgttaaccaccatcaaacaggattttcgcctgctggggcaaaccagcgtggaccgcttgctgcaactctctcagggccaggcggtgaagggcaatcagctgttgcccgtctcactggtgaaaagaaaaaccaccctggcgcccaatacgcaaaccgcctctccccgcgcgttggccgattcattaatgcagctggcacgacaggtttcccgactggaaagcgggcagtgagcgcaacgcaattaatgtaagttagctcactcattaggcaccgggatctcgaccgatgcccttgagagccttcaacccagtcagctccttccggtgggcgcggggcatgactatcgtcgccgcacttatgactgtcttctttatcatgcaactcgtaggacaggtgccggcagcgctctgggtcattttcggcgaggaccgctttcgctggagcgcgacgatgatcggcctgtcgcttgcggtattcggaatcttgcacgccctcgctcaagccttcgtcactggtcccgccaccaaacgtttcggcgagaagcaggccattatcgccggcatggcggccccacgggtgcgcatgatcgtgctcctgtcgttgaggacccggctaggctggcggggttgccttactggttagcagaatgaatcaccgatacgcgagcgaacgtgaagcgactgctgctgcaaaacgtctgcgacctgagcaacaacatgaatggtcttcggtttccgtgtttcgtaaagtctggaaacgcggaagtcagcgccctgcaccattatgttccggatctgcatcgcaggatgctgctggctaccctgtggaacacctacatctgtattaacgaagcgctggcattgaccctgagtgatttttctctggtcccgccgcatccataccgccagttgtttaccctcacaacgttccagtaaccgggcatgttcatcatcagtaacccgtatcgtgagcatcctctctcgtttcatcggtatcattacccccatgaacagaaatcccccttacacggaggcatcagtgaccaaacaggaaaaaaccgcccttaacatggcccgctttatcagaagccagacattaacgcttctggagaaactcaacgagctggacgcggatgaacaggcagacatctgtgaatcgcttcacgaccacgctgatgagctttaccgcagctgcctcgcgcgtttcggtgatgacggtgaaaacctctgacacatgcagctcccggagacggtcacagcttgtctgtaagcggatgccgggagcagacaagcccgtcagggcgcgtcagcgggtgttggcgggtgtcggggcgcagccatgacccagtcacgtagcgatagcggagtgtatactggcttaactatgcggcatcagagcagattgtactgagagtgcaccatatatgcggtgtgaaataccgcacagatgcgtaaggagaaaataccgcatcaggcgctcttccgcttcctcgctcactgactcgctgcgctcggtcgttcggctgcggcgagcggtatcagctcactcaaaggcggtaatacggttatccacagaatcaggggataacgcaggaaagaacatgtgagcaaaaggccagcaaaaggccaggaaccgtaaaaaggccgcgttgctggcgtttttccataggctccgcccccctgacgagcatcacaaaaatcgacgctcaagtcagaggtggcgaaacccgacaggactataaagataccaggcgtttccccctggaagctccctcgtgcgctctcctgttccgaccctgccgcttaccggatacctgtccgcctttctcccttcgggaagcgtggcgctttctcatagctcacgctgtaggtatctcagttcggtgtaggtcgttcgctccaagctgggctgtgtgcacgaaccccccgttcagcccgaccgctgcgccttatccggtaactatcgtcttgagtccaacccggtaagacacgacttatcgccactggcagcagccactggtaacaggattagcagagcgaggtatgtaggcggtgctacagagttcttgaagtggtggcctaactacggctacactagaaggacagtatttggtatctgcgctctgctgaagccagttaccttcggaaaaagagttggtagctcttgatccggcaaacaaaccaccgctggtagcggtggtttttttgtttgcaagcagcagattacgcgcagaaaaaaaggatctcaagaagatcctttgatcttttctacggggtctgacgctcagtggaacgaaaactcacgttaagggattttggtcatgagattatcaaaaaggatcttcacctagatccttttaaattaaaaatgaagttttaaatcaatctaaagtatatatgagtaaacttggtctgacagttaccaatgcttaatcagtgaggcacctatctcagcgatctgtctatttcgttcatccatagttgcctgactccccgtcgtgtagataactacgatacgggagggcttaccatctggccccagtgctgcaatgataccgcgagacccacgctcaccggctccagatttatcagcaataaaccagccagccggaagggccgagcgcagaagtggtcctgcaactttatccgcctccatccagtctattaattgttgccgggaagctagagtaagtagttcgccagttaatagtttgcgcaacgttgttgccattgctgcaggcatcgtggtgtcacgctcgtcgtttggtatggcttcattcagctccggttcccaacgatcaaggcgagttacatgatcccccatgttgtgcaaaaaagcggttagctccttcggtcctccgatcgttgtcagaagtaagttggccgcagtgttatcactcatggttatggcagcactgcataattctcttactgtcatgccatccgtaagatgcttttctgtgactggtgagtactcaaccaagtcattctgagaatagtgtatgcggcgaccgagttgctcttgcccggcgtcaatacgggataataccgcgccacatagcagaactttaaaagtgctcatcattggaaaacgttcttcggggcgaaaactctcaaggatcttaccgctgttgagatccagttcgatgtaacccactcgtgcacccaactgatcttcagcatcttttactttcaccagcgtttctgggtgagcaaaaacaggaaggcaaaatgccgcaaaaaagggaataagggcgacacggaaatgttgaatactcatactcttcctttttcaatattattgaagcatttatcagggttattgtctcatgagcggatacatatttgaatgtatttagaaaaataaacaaataggggttccgcgcacatttccccgaaaagtgccacctgaaattgtaaacgttaatattttgttaaaattcgcgttaaatttttgttaaatcagctcattttttaaccaataggccgaaatcggcaaaatcccttataaatcaaaagaatagaccgagatagggttgagtgttgttccagtttggaacaagagtccactattaaagaacgtggactccaacgtcaaagggcgaaaaaccgtctatcagggcgatggcccactacgtgaaccatcaccctaatcaagttttttggggtcgaggtgccgtaaagcactaaatcggaaccctaaagggagcccccgatttagagcttgacggggaaagccggcgaacgtggcgagaaaggaagggaagaaagcgaaaggagcgggcgctagggcgctggcaagtgtagcggtcacgctgcgcgtaaccaccacacccgccgcgcttaatgcgccgctacagggcgcgtcccattcgcca

SEQ ID NO: 69 - DNA, 7386 bp, artificial
  pFr3
atccggatatagttcctcctttcagcaaaaaacccctcaagacccgtttagaggccccaaggggttatgctagttattgctcagcggtggcagcagccaactcagcttcctttcgggctttgttagcagccggatctcagtggtggtggtggtggtgctcgagtgcggccgcaagctttcagaactgtgtcgggcgcatcaccgcatcaatgccgccatcaatgacgatctgcgcgccatgcacatagcttgcggccgggctcatcaaaaaggcgatgaccgacgccatctcggacggctcggcacggcggcccatgggaggaacgaacttggcaatggattcgccatagcgcgggtcctgcaggcccgcctgcagcaagggagtctcggttgcaccgggggcgatggtgttcaggcgcacgccagcctcgccccaggcggcggcgcgtttgcgcacagccaccgtcaaagcattcttgctgcccgcataggccagatttccgccctgctctcccgcatgttcgacaatggcgcgggccttggcttcctcgccggcttccagtgccagcgccagtgggttcttgtcaaaagccagatgcgcggaagccacggacgagatgacgacggctgcgggctgatggccttttttcagcgctggcaaaaaggcatccatcagctcggtcgcgccaaaataattgaccgaaaccacattgccaagcaccttggtctgcggtcccaggccggcgcacagcaccaggccgtccatgcccttgctgcacttcgccagtacatcggcaatcgcctgctttcgaccttcggccgtcgagagatcggcaatcacttccgcatcgcgtatatcgatgcctacgatctggtgaccggccgcctccaggaccttgcgcgtagccgcaccaatgccggtggcgcagccgcttatcacgatgatggacatgtatatctcctttcacgaattctcagccgccttcttgaacttggcggcctcttccgaaccgccggtggcattgcccttcgagtaggaatgcgcgccggtgccggcaagagcgccgccctgcacgatgaggtattcgtcgcggatcggacggccctcgaagaagcactccaggatctcgcgggtgcccgccgcataacgcgcctgcgcggtcagcgtggtgccggagatgtgcggggtcatgccgttatagggcatcgtccgccaggggtggtccttcggcgccggctgcgggaaccacacgtcgccggcatagccggccagccggccggattcgagcgcacgtgccacggcatcgcggtcgcacagcttgccgcgggcggtgttgacgatgtaggcgccacgcttgaacagcttcagcgtctcgtcattgatcatgtgctcggtttcggggtgcagcgggcagttcagcgtcaccacgtcgcaaaccggatacatgtcctcgcgggtcgcgtgccaggtgaggttgagctccttctcgaccgattccggcaggcggtgacggtcggtgtagtgcaggtgcacgtcgaacggcgccagacggcgcagcaccgcgagaccgatgcggccggcggccacggtgccgacatgcatcgcctcgaggtcgtaggcgtgggagacgcagtcggcgatgttccagccgcccttccgcgcccattcgtgcgagggcagatagttgcgcaccagcgacaggatcatcatcaccacatgctcggcgacgctgatcgagttgcagtaggtgacttccgccacggtgacgttgcggtcgatagccgactgaagatcgacgtggtcggaaccgatgccggcggtgagcgcgagcttcaggttcttggccttggcgatgcgctcgggcgtcagataggccggccagaagggctgggagatgacgacatccgcatcgaccagctcgcgctcgaacaccgagtcggggccgtccttgtcggaggtcacgaccagggtgtggccgttggattcgagatattcgcgcaggccgagctcgccggagacggagccgagcaactgcccgggcgtgaagtcgatggccttcggcgtcggcaagatctggccgcccggatagtggtcgatcttcggaagatcgtcgcgggcataggtcttcgggtagccgtcgaccggatcatcgtaaagaacgcacaggacctttgccatcatatgtatatctccttcttaaagttaaacaaaattatttctagaggggaattgttatccgctcacaattcccctatagtgagtcgtattaatttcgcgggatcgagatctcgatcctctacgccggacgcatcgtggccggcatcaccggcgccacaggtgcggttgctggcgcctatatcgccgacatcaccgatggggaagatcgggctcgccacttcgggctcatgagcgcttgtttcggcgtgggtatggtggcaggccccgtggccgggggactgttgggcgccatctccttgcatgcaccattccttgcggcggcggtgctcaacggcctcaacctactactgggctgcttcctaatgcaggagtcgcataagggagagcgtcgagatcccggacaccatcgaatggcgcaaaacctttcgcggtatggcatgatagcgcccggaagagagtcaattcagggtggtgaatgtgaaaccagtaacgttatacgatgtcgcagagtatgccggtgtctcttatcagaccgtttcccgcgtggtgaaccaggccagccacgtttctgcgaaaacgcgggaaaaagtggaagcggcgatggcggagctgaattacattcccaaccgcgtggcacaacaactggcgggcaaacagtcgttgctgattggcgttgccacctccagtctggccctgcacgcgccgtcgcaaattgtcgcggcgattaaatctcgcgccgatcaactgggtgccagcgtggtggtgtcgatggtagaacgaagcggcgtcgaagcctgtaaagcggcggtgcacaatcttctcgcgcaacgcgtcagtgggctgatcattaactatccgctggatgaccaggatgccattgctgtggaagctgcctgcactaatgttccggcgttatttcttgatgtctctgaccagacacccatcaacagtattattttctcccatgaagacggtacgcgactgggcgtggagcatctggtcgcattgggtcaccagcaaatcgcgctgttagcgggcccattaagttctgtctcggcgcgtctgcgtctggctggctggcataaatatctcactcgcaatcaaattcagccgatagcggaacgggaaggcgactggagtgccatgtccggttttcaacaaaccatgcaaatgctgaatgagggcatcgttcccactgcgatgctggttgccaacgatcagatggcgctgggcgcaatgcgcgccattaccgagtccgggctgcgcgttggtgcggatatctcggtagtgggatacgacgataccgaagacagctcatgttatatcccgccgttaaccaccatcaaacaggattttcgcctgctggggcaaaccagcgtggaccgcttgctgcaactctctcagggccaggcggtgaagggcaatcagctgttgcccgtctcactggtgaaaagaaaaaccaccctggcgcccaatacgcaaaccgcctctccccgcgcgttggccgattcattaatgcagctggcacgacaggtttcccgactggaaagcgggcagtgagcgcaacgcaattaatgtaagttagctcactcattaggcaccgggatctcgaccgatgcccttgagagccttcaacccagtcagctccttccggtgggcgcggggcatgactatcgtcgccgcacttatgactgtcttctttatcatgcaactcgtaggacaggtgccggcagcgctctgggtcattttcggcgaggaccgctttcgctggagcgcgacgatgatcggcctgtcgcttgcggtattcggaatcttgcacgccctcgctcaagccttcgtcactggtcccgccaccaaacgtttcggcgagaagcaggccattatcgccggcatggcggccccacgggtgcgcatgatcgtgctcctgtcgttgaggacccggctaggctggcggggttgccttactggttagcagaatgaatcaccgatacgcgagcgaacgtgaagcgactgctgctgcaaaacgtctgcgacctgagcaacaacatgaatggtcttcggtttccgtgtttcgtaaagtctggaaacgcggaagtcagcgccctgcaccattatgttccggatctgcatcgcaggatgctgctggctaccctgtggaacacctacatctgtattaacgaagcgctggcattgaccctgagtgatttttctctggtcccgccgcatccataccgccagttgtttaccctcacaacgttccagtaaccgggcatgttcatcatcagtaacccgtatcgtgagcatcctctctcgtttcatcggtatcattacccccatgaacagaaatcccccttacacggaggcatcagtgaccaaacaggaaaaaaccgcccttaacatggcccgctttatcagaagccagacattaacgcttctggagaaactcaacgagctggacgcggatgaacaggcagacatctgtgaatcgcttcacgaccacgctgatgagctttaccgcagctgcctcgcgcgtttcggtgatgacggtgaaaacctctgacacatgcagctcccggagacggtcacagcttgtctgtaagcggatgccgggagcagacaagcccgtcagggcgcgtcagcgggtgttggcgggtgtcggggcgcagccatgacccagtcacgtagcgatagcggagtgtatactggcttaactatgcggcatcagagcagattgtactgagagtgcaccatatatgcggtgtgaaataccgcacagatgcgtaaggagaaaataccgcatcaggcgctcttccgcttcctcgctcactgactcgctgcgctcggtcgttcggctgcggcgagcggtatcagctcactcaaaggcggtaatacggttatccacagaatcaggggataacgcaggaaagaacatgtgagcaaaaggccagcaaaaggccaggaaccgtaaaaaggccgcgttgctggcgtttttccataggctccgcccccctgacgagcatcacaaaaatcgacgctcaagtcagaggtggcgaaacccgacaggactataaagataccaggcgtttccccctggaagctccctcgtgcgctctcctgttccgaccctgccgcttaccggatacctgtccgcctttctcccttcgggaagcgtggcgctttctcatagctcacgctgtaggtatctcagttcggtgtaggtcgttcgctccaagctgggctgtgtgcacgaaccccccgttcagcccgaccgctgcgccttatccggtaactatcgtcttgagtccaacccggtaagacacgacttatcgccactggcagcagccactggtaacaggattagcagagcgaggtatgtaggcggtgctacagagttcttgaagtggtggcctaactacggctacactagaaggacagtatttggtatctgcgctctgctgaagccagttaccttcggaaaaagagttggtagctcttgatccggcaaacaaaccaccgctggtagcggtggtttttttgtttgcaagcagcagattacgcgcagaaaaaaaggatctcaagaagatcctttgatcttttctacggggtctgacgctcagtggaacgaaaactcacgttaagggattttggtcatgagattatcaaaaaggatcttcacctagatccttttaaattaaaaatgaagttttaaatcaatctaaagtatatatgagtaaacttggtctgacagttaccaatgcttaatcagtgaggcacctatctcagcgatctgtctatttcgttcatccatagttgcctgactccccgtcgtgtagataactacgatacgggagggcttaccatctggccccagtgctgcaatgataccgcgagacccacgctcaccggctccagatttatcagcaataaaccagccagccggaagggccgagcgcagaagtggtcctgcaactttatccgcctccatccagtctattaattgttgccgggaagctagagtaagtagttcgccagttaatagtttgcgcaacgttgttgccattgctgcaggcatcgtggtgtcacgctcgtcgtttggtatggcttcattcagctccggttcccaacgatcaaggcgagttacatgatcccccatgttgtgcaaaaaagcggttagctccttcggtcctccgatcgttgtcagaagtaagttggccgcagtgttatcactcatggttatggcagcactgcataattctcttactgtcatgccatccgtaagatgcttttctgtgactggtgagtactcaaccaagtcattctgagaatagtgtatgcggcgaccgagttgctcttgcccggcgtcaatacgggataataccgcgccacatagcagaactttaaaagtgctcatcattggaaaacgttcttcggggcgaaaactctcaaggatcttaccgctgttgagatccagttcgatgtaacccactcgtgcacccaactgatcttcagcatcttttactttcaccagcgtttctgggtgagcaaaaacaggaaggcaaaatgccgcaaaaaagggaataagggcgacacggaaatgttgaatactcatactcttcctttttcaatattattgaagcatttatcagggttattgtctcatgagcggatacatatttgaatgtatttagaaaaataaacaaataggggttccgcgcacatttccccgaaaagtgccacctgaaattgtaaacgttaatattttgttaaaattcgcgttaaatttttgttaaatcagctcattttttaaccaataggccgaaatcggcaaaatcccttataaatcaaaagaatagaccgagatagggttgagtgttgttccagtttggaacaagagtccactattaaagaacgtggactccaacgtcaaagggcgaaaaaccgtctatcagggcgatggcccactacgtgaaccatcaccctaatcaagttttttggggtcgaggtgccgtaaagcactaaatcggaaccctaaagggagcccccgatttagagcttgacggggaaagccggcgaacgtggcgagaaaggaagggaagaaagcgaaaggagcgggcgctagggcgctggcaagtgtagcggtcacgctgcgcgtaaccaccacacccgccgcgcttaatgcgccgctacagggcgcgtcccattcgcca